European Patent Application EP 4 201 954 A1, published June 28, 2023. Title: Proteins and T-cells involved in chronic inflammatory diseases. Applicant: Christian-Albrechts-Universität zu Kiel. The sequence listing filed with the application follows.

SEQUENCE LISTING (1205 sequences)

SEQ ID NO: 1 - protein, 15 aa, Homo sapiens
  misc_feature (4)..(5): Xaa can be any naturally occurring amino acid
  misc_feature (7)..(7): Xaa can be any naturally occurring amino acid
CVVXXAXGGSYIPTF

SEQ ID NO: 2 - protein, 15 aa, Homo sapiens
CVVNLASGGSYIPTF

SEQ ID NO: 3 - protein, 15 aa, Homo sapiens
CVVNGASGGSYIPTF

SEQ ID NO: 4 - protein, 15 aa, Homo sapiens
CVVNSASGGSYIPTF

SEQ ID NO: 5 - protein, 15 aa, Homo sapiens
CVVNIASGGSYIPTF

SEQ ID NO: 6 - protein, 15 aa, Homo sapiens
CVVNPASGGSYIPTF

SEQ ID NO: 7 - protein, 15 aa, Homo sapiens
CVVNRASGGSYIPTF

SEQ ID NO: 8 - protein, 15 aa, Homo sapiens
CVVSLASGGSYIPTF

SEQ ID NO: 9 - protein, 15 aa, Homo sapiens
CVVNMASGGSYIPTF

SEQ ID NO: 10 - protein, 15 aa, Homo sapiens
CVVTLASGGSYIPTF

SEQ ID NO: 11 - protein, 15 aa, Homo sapiens
CVVNTASGGSYIPTF

SEQ ID NO: 12 - protein, 15 aa, Homo sapiens
CVVRLASGGSYIPTF

SEQ ID NO: 13 - protein, 15 aa, Homo sapiens
CVVRHASGGSYIPTF

SEQ ID NO: 14 - protein, 15 aa, Homo sapiens
CVVNVASGGSYIPTF

SEQ ID NO: 15 - protein, 15 aa, Homo sapiens
CVVSHASGGSYIPTF

SEQ ID NO: 16 - protein, 15 aa, Homo sapiens
CVVRVASGGSYIPTF

SEQ ID NO: 17 - protein, 15 aa, Homo sapiens
CVVRSASGGSYIPTF

SEQ ID NO: 18 - protein, 15 aa, Homo sapiens
CVVIPASGGSYIPTF

SEQ ID NO: 19 - protein, 15 aa, Homo sapiens
CVVNKASGGSYIPTF

SEQ ID NO: 20 - protein, 15 aa, Homo sapiens
CVVRGASGGSYIPTF

SEQ ID NO: 21 - protein, 15 aa, Homo sapiens
CVVTPASGGSYIPTF

SEQ ID NO: 22 - protein, 15 aa, Homo sapiens
CVVNAASGGSYIPTF

SEQ ID NO: 23 - protein, 15 aa, Homo sapiens
CVVNFASGGSYIPTF

SEQ ID NO: 24 - protein, 15 aa, Homo sapiens
CVVSSASGGSYIPTF

SEQ ID NO: 25 - protein, 15 aa, Homo sapiens
CVVNQASGGSYIPTF

SEQ ID NO: 26 - protein, 15 aa, Homo sapiens
CVVRTASGGSYIPTF

SEQ ID NO: 27 - protein, 15 aa, Homo sapiens
CVVIHASGGSYIPTF

SEQ ID NO: 28 - protein, 15 aa, Homo sapiens
CVVNEASGGSYIPTF

SEQ ID NO: 29 - protein, 15 aa, Homo sapiens
CVVNHASGGSYIPTF

SEQ ID NO: 30 - protein, 15 aa, Homo sapiens
CVVRRASGGSYIPTF

SEQ ID NO: 31 - protein, 15 aa, Homo sapiens
CVVILASGGSYIPTF

SEQ ID NO: 32 - protein, 15 aa, Homo sapiens
CVVRIASGGSYIPTF

SEQ ID NO: 33 - protein, 15 aa, Homo sapiens
CVVRAASGGSYIPTF

SEQ ID NO: 34 - protein, 15 aa, Homo sapiens
CVVSPASGGSYIPTF

SEQ ID NO: 35 - protein, 15 aa, Homo sapiens
CVVSTASGGSYIPTF

SEQ ID NO: 36 - protein, 15 aa, Homo sapiens
CVVTHASGGSYIPTF

SEQ ID NO: 37 - protein, 15 aa, Homo sapiens
CVVTSASGGSYIPTF

SEQ ID NO: 38 - protein, 15 aa, Homo sapiens
CVVTVASGGSYIPTF

SEQ ID NO: 39 - protein, 15 aa, Homo sapiens
CVVNMAAGGSYIPTF

SEQ ID NO: 40 - protein, 15 aa, Homo sapiens
CVVSVASGGSYIPTF

SEQ ID NO: 41 - protein, 15 aa, Homo sapiens
CVVTAASGGSYIPTF

SEQ ID NO: 42 - protein, 15 aa, Homo sapiens
CVVKGASGGSYIPTF

SEQ ID NO: 43 - protein, 15 aa, Homo sapiens
CVVNGAPGGSYIPTF

SEQ ID NO: 44 - protein, 15 aa, Homo sapiens
CVVNIAAGGSYIPTF

SEQ ID NO: 45 - protein, 15 aa, Homo sapiens
CVVNMATGGSYIPTF

SEQ ID NO: 46 - protein, 15 aa, Homo sapiens
CVVPHASGGSYIPTF

SEQ ID NO: 47 - protein, 15 aa, Homo sapiens
CVVSAASGGSYIPTF

SEQ ID NO: 48 - protein, 15 aa, Homo sapiens
CVVTFASGGSYIPTF

SEQ ID NO: 49 - protein, 15 aa, Homo sapiens
CVVREASGGSYIPTF

SEQ ID NO: 50 - protein, 15 aa, Homo sapiens
CVVSFASGGSYIPTF

SEQ ID NO: 51 - protein, 15 aa, Homo sapiens
CVVSGASGGSYIPTF

SEQ ID NO: 52 - protein, 15 aa, Homo sapiens
CVVSIASGGSYIPTF

SEQ ID NO: 53 - protein, 15 aa, Homo sapiens
CVVIAASGGSYIPTF

SEQ ID NO: 54 - protein, 15 aa, Homo sapiens
CVVISASGGSYIPTF

SEQ ID NO: 55 - protein, 15 aa, Homo sapiens
CVVNMAGGGSYIPTF

SEQ ID NO: 56 - protein, 15 aa, Homo sapiens
CVVFHASGGSYIPTF

SEQ ID NO: 57 - protein, 15 aa, Homo sapiens
CVVRQASGGSYIPTF

SEQ ID NO: 58 - protein, 15 aa, Homo sapiens
CVVSRASGGSYIPTF

SEQ ID NO: 59 - protein, 15 aa, Homo sapiens
CVVIGASGGSYIPTF

SEQ ID NO: 60 - protein, 15 aa, Homo sapiens
CVVLHASGGSYIPTF

SEQ ID NO: 61 - protein, 15 aa, Homo sapiens
CVVNIATGGSYIPTF

SEQ ID NO: 62 - protein, 15 aa, Homo sapiens
CVVNYASGGSYIPTF

SEQ ID NO: 63 - protein, 15 aa, Homo sapiens
CVVRFASGGSYIPTF

SEQ ID NO: 64 - protein, 15 aa, Homo sapiens
CVVTLAGGGSYIPTF

SEQ ID NO: 65 - protein, 15 aa, Homo sapiens
CVVAHASGGSYIPTF

SEQ ID NO: 66 - protein, 15 aa, Homo sapiens
CVVIRASGGSYIPTF

SEQ ID NO: 67 - protein, 15 aa, Homo sapiens
CVVNGAAGGSYIPTF

SEQ ID NO: 68 - protein, 15 aa, Homo sapiens
CVVNIAGGGSYIPTF

SEQ ID NO: 69 - protein, 15 aa, Homo sapiens
CVVRMASGGSYIPTF

SEQ ID NO: 70 - protein, 15 aa, Homo sapiens
CVVTIASGGSYIPTF

SEQ ID NO: 71 - protein, 15 aa, Homo sapiens
CVVKHASGGSYIPTF

SEQ ID NO: 72 - protein, 15 aa, Homo sapiens
CVVKSASGGSYIPTF

SEQ ID NO: 73 - protein, 15 aa, Homo sapiens
CVVMGASGGSYIPTF

SEQ ID NO: 74 - protein, 15 aa, Homo sapiens
CVVNDASGGSYIPTF

SEQ ID NO: 75 - protein, 15 aa, Homo sapiens
CVVNRAPGGSYIPTF

SEQ ID NO: 76 - protein, 15 aa, Homo sapiens
CVVTGASGGSYIPTF

SEQ ID NO: 77 - protein, 15 aa, Homo sapiens
CVVALASGGSYIPTF

SEQ ID NO: 78 - protein, 15 aa, Homo sapiens
CVVDHASGGSYIPTF

SEQ ID NO: 79 - protein, 15 aa, Homo sapiens
CVVIFASGGSYIPTF

SEQ ID NO: 80 - protein, 15 aa, Homo sapiens
CVVIIASGGSYIPTF

SEQ ID NO: 81 - protein, 15 aa, Homo sapiens
CVVIVASGGSYIPTF

SEQ ID NO: 82 - protein, 15 aa, Homo sapiens
CVVKPASGGSYIPTF

SEQ ID NO: 83 - protein, 15 aa, Homo sapiens
CVVKRASGGSYIPTF

SEQ ID NO: 84 - protein, 15 aa, Homo sapiens
CVVKTASGGSYIPTF

SEQ ID NO: 85 - protein, 15 aa, Homo sapiens
CVVNLAAGGSYIPTF

SEQ ID NO: 86 - protein, 15 aa, Homo sapiens
CVVNSAAGGSYIPTF

SEQ ID NO: 87 - protein, 15 aa, Homo sapiens
CVVNSAGGGSYIPTF

SEQ ID NO: 88 - protein, 15 aa, Homo sapiens
CVVRKASGGSYIPTF

SEQ ID NO: 89 - protein, 15 aa, Homo sapiens
CVVSQASGGSYIPTF

SEQ ID NO: 90 - protein, 15 aa, Homo sapiens
CVVFLASGGSYIPTF

SEQ ID NO: 91 - protein, 15 aa, Homo sapiens
CVVFSASGGSYIPTF

SEQ ID NO: 92 - protein, 15 aa, Homo sapiens
CVVKAASGGSYIPTF

SEQ ID NO: 93 - protein, 15 aa, Homo sapiens
CVVKLASGGSYIPTF

SEQ ID NO: 94 - protein, 15 aa, Homo sapiens
CVVMHASGGSYIPTF

SEQ ID NO: 95 - protein, 15 aa, Homo sapiens
CVVNLAGGGSYIPTF

SEQ ID NO: 96 - protein, 15 aa, Homo sapiens
CVVNMAPGGSYIPTF

SEQ ID NO: 97 - protein, 15 aa, Homo sapiens
CVVNRAAGGSYIPTF

SEQ ID NO: 98 - protein, 15 aa, Homo sapiens
CVVNRATGGSYIPTF

SEQ ID NO: 99 - protein, 15 aa, Homo sapiens
CVVNVAAGGSYIPTF

SEQ ID NO: 100 - protein, 15 aa, Homo sapiens
CVVNVATGGSYIPTF

SEQ ID NO: 101 - protein, 15 aa, Homo sapiens
CVVNWASGGSYIPTF

SEQ ID NO: 102 - protein, 15 aa, Homo sapiens
CVVSKASGGSYIPTF

SEQ ID NO: 103 - protein, 15 aa, Homo sapiens
CVVSQAAGGSYIPTF

SEQ ID NO: 104 - protein, 15 aa, Homo sapiens
CVVTDASGGSYIPTF

SEQ ID NO: 105 - protein, 15 aa, Homo sapiens
CVVTYASGGSYIPTF

SEQ ID NO: 106 - protein, 15 aa, Homo sapiens
CVVGLASGGSYIPTF

SEQ ID NO: 107 - protein, 15 aa, Homo sapiens
CVVGTASGGSYIPTF

SEQ ID NO: 108 - protein, 15 aa, Homo sapiens
CVVIDASGGSYIPTF

SEQ ID NO: 109 - protein, 15 aa, Homo sapiens
CVVITASGGSYIPTF

SEQ ID NO: 110 - protein, 15 aa, Homo sapiens
CVVKVASGGSYIPTF

SEQ ID NO: 111 - protein, 15 aa, Homo sapiens
CVVLLASGGSYIPTF

SEQ ID NO: 112 - protein, 15 aa, Homo sapiens
CVVNGATGGSYIPTF

SEQ ID NO: 113 - protein, 15 aa, Homo sapiens
CVVNIAPGGSYIPTF

SEQ ID NO: 114 - protein, 15 aa, Homo sapiens
CVVNKAAGGSYIPTF

SEQ ID NO: 115 - protein, 15 aa, Homo sapiens
CVVNLARGGSYIPTF

SEQ ID NO: 116 - protein, 15 aa, Homo sapiens
CVVNSAVGGSYIPTF

SEQ ID NO: 117 - protein, 15 aa, Homo sapiens
CVVNTAGGGSYIPTF

SEQ ID NO: 118 - protein, 15 aa, Homo sapiens
CVVNVAGGGSYIPTF

SEQ ID NO: 119 - protein, 15 aa, Homo sapiens
CVVTQASGGSYIPTF

SEQ ID NO: 120 - protein, 15 aa, Homo sapiens
CVVTTASGGSYIPTF

SEQ ID NO: 121 - protein, 15 aa, Homo sapiens
CVVYHASGGSYIPTF

SEQ ID NO: 122 - protein, 15 aa, Homo sapiens
CVVYLASGGSYIPTF

SEQ ID NO: 123 - protein, 15 aa, Homo sapiens
CVVADASGGSYIPTF

SEQ ID NO: 124 - protein, 15 aa, Homo sapiens
CVVAQASGGSYIPTF

SEQ ID NO: 125 - protein, 15 aa, Homo sapiens
CVVASASGGSYIPTF

SEQ ID NO: 126 - protein, 15 aa, Homo sapiens
CVVATASGGSYIPTF

SEQ ID NO: 127 - protein, 15 aa, Homo sapiens
CVVFGASGGSYIPTF

SEQ ID NO: 128 - protein, 15 aa, Homo sapiens
CVVHHASGGSYIPTF

SEQ ID NO: 129 - protein, 15 aa, Homo sapiens
CVVHVASGGSYIPTF

SEQ ID NO: 130 - protein, 15 aa, Homo sapiens
CVVINASGGSYIPTF

SEQ ID NO: 131 - protein, 15 aa, Homo sapiens
CVVIQASGGSYIPTF

SEQ ID NO: 132 - protein, 15 aa, Homo sapiens
CVVKEASGGSYIPTF

SEQ ID NO: 133 - protein, 15 aa, Homo sapiens
CVVKIASGGSYIPTF

SEQ ID NO: 134 - protein, 15 aa, Homo sapiens
CVVKKASGGSYIPTF

SEQ ID NO: 135 - protein, 15 aa, Homo sapiens
CVVKMASGGSYIPTF

SEQ ID NO: 136 - protein, 15 aa, Homo sapiens
CVVKRAGGGSYIPTF

SEQ ID NO: 137 - protein, 15 aa, Homo sapiens
CVVLGASGGSYIPTF

SEQ ID NO: 138 - protein, 15 aa, Homo sapiens
CVVLPASGGSYIPTF

SEQ ID NO: 139 - protein, 15 aa, Homo sapiens
CVVLSASGGSYIPTF

SEQ ID NO: 140 - protein, 15 aa, Homo sapiens
CVVLTASGGSYIPTF

SEQ ID NO: 141 - protein, 15 aa, Homo sapiens
CVVMPASGGSYIPTF

SEQ ID NO: 142 - protein, 15 aa, Homo sapiens
CVVNEAAGGSYIPTF

SEQ ID NO: 143 - protein, 15 aa, Homo sapiens
CVVNIALGGSYIPTF

SEQ ID NO: 144 - protein, 15 aa, Homo sapiens
CVVNIARGGSYIPTF

SEQ ID NO: 145 - protein, 15 aa, Homo sapiens
CVVNMAEGGSYIPTF

SEQ ID NO: 146 - protein, 15 aa, Homo sapiens
CVVNPATGGSYIPTF

SEQ ID NO: 147 - protein, 15 aa, Homo sapiens
CVVNSATGGSYIPTF

SEQ ID NO: 148 - protein, 15 aa, Homo sapiens
CVVPFASGGSYIPTF

SEQ ID NO: 149 - protein, 15 aa, Homo sapiens
CVVPPASGGSYIPTF

SEQ ID NO: 150 - protein, 15 aa, Homo sapiens
CVVPRASGGSYIPTF

SEQ ID NO: 151 - protein, 15 aa, Homo sapiens
CVVPSASGGSYIPTF

SEQ ID NO: 152 - protein, 15 aa, Homo sapiens
CVVPTASGGSYIPTF

SEQ ID NO: 153 - protein, 15 aa, Homo sapiens
CVVRLAGGGSYIPTF

SEQ ID NO: 154 - protein, 15 aa, Homo sapiens
CVVRPASGGSYIPTF

SEQ ID NO: 155 - protein, 15 aa, Homo sapiens
CVVRTARGGSYIPTF

SEQ ID NO: 156 - protein, 15 aa, Homo sapiens
CVVRVAAGGSYIPTF

SEQ ID NO: 157 - protein, 15 aa, Homo sapiens
CVVRYASGGSYIPTF

SEQ ID NO: 158 - protein, 15 aa, Homo sapiens
CVVSDASGGSYIPTF

SEQ ID NO: 159 - protein, 15 aa, Homo sapiens
CVVSGAVGGSYIPTF

SEQ ID NO: 160 - protein, 15 aa, Homo sapiens
CVVSLAGGGSYIPTF

SEQ ID NO: 161 - protein, 15 aa, Homo sapiens
CVVVHASGGSYIPTF

SEQ ID NO: 162 - protein, 15 aa, Homo sapiens
CVVVLASGGSYIPTF

SEQ ID NO: 163 - protein, 15 aa, Homo sapiens
CVVAFASGGSYIPTF

SEQ ID NO: 164 - protein, 15 aa, Homo sapiens
CVVAGASGGSYIPTF

SEQ ID NO: 165 - protein, 15 aa, Homo sapiens
CVVAPASGGSYIPTF

SEQ ID NO: 166 - protein, 15 aa, Homo sapiens
CVVAVASGGSYIPTF

SEQ ID NO: 167 - protein, 15 aa, Homo sapiens
CVVAWASGGSYIPTF

SEQ ID NO: 168 - protein, 15 aa, Homo sapiens
CVVDDASGGSYIPTF

SEQ ID NO: 169 - protein, 15 aa, Homo sapiens
CVVDQASGGSYIPTF

SEQ ID NO: 170 - protein, 15 aa, Homo sapiens
CVVEQASGGSYIPTF

SEQ ID NO: 171 - protein, 15 aa, Homo sapiens
CVVFAASGGSYIPTF

SEQ ID NO: 172 - protein, 15 aa, Homo sapiens
CVVFLAGGGSYIPTF

SEQ ID NO: 173 - protein, 15 aa, Homo sapiens
CVVFQARGGSYIPTF

SEQ ID NO: 174 - protein, 15 aa, Homo sapiens
CVVFQASGGSYIPTF

SEQ ID NO: 175 - protein, 15 aa, Homo sapiens
CVVFRASGGSYIPTF

SEQ ID NO: 176 - protein, 15 aa, Homo sapiens
CVVFTASGGSYIPTF

SEQ ID NO: 177 - protein, 15 aa, Homo sapiens
CVVFVASGGSYIPTF

SEQ ID NO: 178 - protein, 15 aa, Homo sapiens
CVVGDASGGSYIPTF

SEQ ID NO: 179 - protein, 15 aa, Homo sapiens
CVVGIASGGSYIPTF

SEQ ID NO: 180 - protein, 15 aa, Homo sapiens
CVVGRASGGSYIPTF

SEQ ID NO: 181 - protein, 15 aa, Homo sapiens
CVVGVAAGGSYIPTF

SEQ ID NO: 182 - protein, 15 aa, Homo sapiens
CVVGVASGGSYIPTF

SEQ ID NO: 183 - protein, 15 aa, Homo sapiens
CVVHDASGGSYIPTF

SEQ ID NO: 184 - protein, 15 aa, Homo sapiens
CVVHEASGGSYIPTF

SEQ ID NO: 185 - protein, 15 aa, Homo sapiens
CVVHLASGGSYIPTF

SEQ ID NO: 186 - protein, 15 aa, Homo sapiens
CVVHQASGGSYIPTF

SEQ ID NO: 187 - protein, 15 aa, Homo sapiens
CVVHYASGGSYIPTF

SEQ ID NO: 188 - protein, 15 aa, Homo sapiens
CVVIPATGGSYIPTF

SEQ ID NO: 189 - protein, 15 aa, Homo sapiens
CVVISAPGGSYIPTF

SEQ ID NO: 190 - protein, 15 aa, Homo sapiens
CVVIYASGGSYIPTF

SEQ ID NO: 191 - protein, 15 aa, Homo sapiens
CVVKAAAGGSYIPTF

SEQ ID NO: 192 - protein, 15 aa, Homo sapiens
CVVKDASGGSYIPTF

SEQ ID NO: 193 - protein, 15 aa, Homo sapiens
CVVKFASGGSYIPTF

SEQ ID NO: 194 - protein, 15 aa, Homo sapiens
CVVKGAGGGSYIPTF

SEQ ID NO: 195 - protein, 15 aa, Homo sapiens
CVVKGAPGGSYIPTF

SEQ ID NO: 196 - protein, 15 aa, Homo sapiens
CVVKLAVGGSYIPTF

SEQ ID NO: 197 - protein, 15 aa, Homo sapiens
CVVKNASGGSYIPTF

SEQ ID NO: 198 - protein, 15 aa, Homo sapiens
CVVKSAGGGSYIPTF

SEQ ID NO: 199 - protein, 15 aa, Homo sapiens
CVVKTAAGGSYIPTF

SEQ ID NO: 200 - protein, 15 aa, Homo sapiens
CVVKTAGGGSYIPTF

SEQ ID NO: 201 - protein, 15 aa, Homo sapiens
CVVKVAGGGSYIPTF

SEQ ID NO: 202 - protein, 15 aa, Homo sapiens
CVVKYASGGSYIPTF

SEQ ID NO: 203 - protein, 15 aa, Homo sapiens
CVVLGAAGGSYIPTF

SEQ ID NO: 204 - protein, 15 aa, Homo sapiens
CVVLVASGGSYIPTF

SEQ ID NO: 205 - protein, 15 aa, Homo sapiens
CVVMAASGGSYIPTF

SEQ ID NO: 206 - protein, 15 aa, Homo sapiens
CVVMKAEGGSYIPTF

SEQ ID NO: 207 - protein, 15 aa, Homo sapiens
CVVMLASGGSYIPTF

SEQ ID NO: 208 - protein, 15 aa, Homo sapiens
CVVMRASGGSYIPTF

SEQ ID NO: 209 - protein, 15 aa, Homo sapiens
CVVMTASGGSYIPTF

SEQ ID NO: 210 - protein, 15 aa, Homo sapiens
CVVNAAAGGSYIPTF

SEQ ID NO: 211 - protein, 15 aa, Homo sapiens
CVVNAAPGGSYIPTF

SEQ ID NO: 212 - protein, 15 aa, Homo sapiens
CVVNAARGGSYIPTF

SEQ ID NO: 213 - protein, 15 aa, Homo sapiens
CVVNAATGGSYIPTF

SEQ ID NO: 214 - protein, 15 aa, Homo sapiens
CVVNEAGGGSYIPTF

SEQ ID NO: 215 - protein, 15 aa, Homo sapiens
CVVNEATGGSYIPTF

SEQ ID NO: 216 - protein, 15 aa, Homo sapiens
CVVNGAGGGSYIPTF

SEQ ID NO: 217 - protein, 15 aa, Homo sapiens
CVVNGAQGGSYIPTF

SEQ ID NO: 218 - protein, 15 aa, Homo sapiens
CVVNGARGGSYIPTF

SEQ ID NO: 219 - protein, 15 aa, Homo sapiens
CVVNGAVGGSYIPTF

SEQ ID NO: 220 - protein, 15 aa, Homo sapiens
CVVNIAEGGSYIPTF

SEQ ID NO: 221 - protein, 15 aa, Homo sapiens
CVVNIAIGGSYIPTF

SEQ ID NO: 222 - protein, 15 aa, Homo sapiens
CVVNKAKGGSYIPTF

SEQ ID NO: 223 - protein, 15 aa, Homo sapiens
CVVNKAPGGSYIPTF

SEQ ID NO: 224 - protein, 15 aa, Homo sapiens
CVVNKATGGSYIPTF

SEQ ID NO: 225 - protein, 15 aa, Homo sapiens
CVVNLAVGGSYIPTF

SEQ ID NO: 226 - protein, 15 aa, Homo sapiens
CVVNMALGGSYIPTF

SEQ ID NO: 227 - protein, 15 aa, Homo sapiens
CVVNMAQGGSYIPTF

SEQ ID NO: 228 - protein, 15 aa, Homo sapiens
CVVNMARGGSYIPTF

SEQ ID NO: 229 - protein, 15 aa, Homo sapiens
CVVNNAPGGSYIPTF

SEQ ID NO: 230 - protein, 15 aa, Homo sapiens
CVVNNARGGSYIPTF

SEQ ID NO: 231 - protein, 15 aa, Homo sapiens
CVVNNASGGSYIPTF

SEQ ID NO: 232 - protein, 15 aa, Homo sapiens
CVVNPALGGSYIPTF

SEQ ID NO: 233 - protein, 15 aa, Homo sapiens
CVVNPAPGGSYIPTF

SEQ ID NO: 234 - protein, 15 aa, Homo sapiens
CVVNQAAGGSYIPTF

SEQ ID NO: 235 - protein, 15 aa, Homo sapiens
CVVNQATGGSYIPTF

SEQ ID NO: 236 - protein, 15 aa, Homo sapiens
CVVNRAGGGSYIPTF

SEQ ID NO: 237 - protein, 15 aa, Homo sapiens
CVVNSAEGGSYIPTF

SEQ ID NO: 238 - protein, 15 aa, Homo sapiens
CVVNSAKGGSYIPTF

SEQ ID NO: 239 - protein, 15 aa, Homo sapiens
CVVNTAAGGSYIPTF

SEQ ID NO: 240 - protein, 15 aa, Homo sapiens
CVVNTAKGGSYIPTF

SEQ ID NO: 241 - protein, 15 aa, Homo sapiens
CVVNTAPGGSYIPTF

SEQ ID NO: 242 - protein, 15 aa, Homo sapiens
CVVNTARGGSYIPTF

SEQ ID NO: 243 - protein, 15 aa, Homo sapiens
CVVNVAPGGSYIPTF

SEQ ID NO: 244 - protein, 15 aa, Homo sapiens
CVVNWAAGGSYIPTF

SEQ ID NO: 245 - protein, 15 aa, Homo sapiens
CVVNWAGGGSYIPTF

SEQ ID NO: 246 - protein, 15 aa, Homo sapiens
CVVPEASGGSYIPTF

SEQ ID NO: 247 - protein, 15 aa, Homo sapiens
CVVPGASGGSYIPTF

SEQ ID NO: 248 - protein, 15 aa, Homo sapiens
CVVPLASGGSYIPTF

SEQ ID NO: 249 - protein, 15 aa, Homo sapiens
CVVPLATGGSYIPTF

SEQ ID NO: 250 - protein, 15 aa, Homo sapiens
CVVPPAPGGSYIPTF

SEQ ID NO: 251 - protein, 15 aa, Homo sapiens
CVVPVASGGSYIPTF

SEQ ID NO: 252 - protein, 15 aa, Homo sapiens
CVVQGASGGSYIPTF

SEQ ID NO: 253 - protein, 15 aa, Homo sapiens
CVVQHASGGSYIPTF

SEQ ID NO: 254 - protein, 15 aa, Homo sapiens
CVVQLASGGSYIPTF

SEQ ID NO: 255 - protein, 15 aa, Homo sapiens
CVVQSASGGSYIPTF

SEQ ID NO: 256 - protein, 15 aa, Homo sapiens
CVVRDASGGSYIPTF

SEQ ID NO: 257 - protein, 15 aa, Homo sapiens
CVVREAWGGSYIPTF

SEQ ID NO: 258 - protein, 15 aa, Homo sapiens
CVVRFARGGSYIPTF

SEQ ID NO: 259 - protein, 15 aa, Homo sapiens
CVVRGAEGGSYIPTF

SEQ ID NO: 260 - protein, 15 aa, Homo sapiens
CVVRHATGGSYIPTF

SEQ ID NO: 261 - protein, 15 aa, Homo sapiens
CVVRQAGGGSYIPTF

SEQ ID NO: 262 - protein, 15 aa, Homo sapiens
CVVRRAAGGSYIPTF

SEQ ID NO: 263 - protein, 15 aa, Homo sapiens
CVVRSATGGSYIPTF

SEQ ID NO: 264 - protein, 15 aa, Homo sapiens
CVVRTAQGGSYIPTF

SEQ ID NO: 265 - protein, 15 aa, Homo sapiens
CVVRVAGGGSYIPTF

SEQ ID NO: 266 - protein, 15 aa, Homo sapiens
CVVSEASGGSYIPTF

SEQ ID NO: 267 - protein, 15 aa, Homo sapiens
CVVSGAQGGSYIPTF

SEQ ID NO: 268 - protein, 15 aa, Homo sapiens
CVVSLAAGGSYIPTF

SEQ ID NO: 269 - protein, 15 aa, Homo sapiens
CVVSLAKGGSYIPTF

SEQ ID NO: 270 - protein, 15 aa, Homo sapiens
CVVSMASGGSYIPTF

SEQ ID NO: 271 - protein, 15 aa, Homo sapiens
CVVSPAPGGSYIPTF

SEQ ID NO: 272 - protein, 15 aa, Homo sapiens
CVVSQAGGGSYIPTF

SEQ ID NO: 273 - protein, 15 aa, Homo sapiens
CVVSRAMGGSYIPTF

SEQ ID NO: 274 - protein, 15 aa, Homo sapiens
CVVSSAVGGSYIPTF

SEQ ID NO: 275 - protein, 15 aa, Homo sapiens
CVVSTATGGSYIPTF

SEQ ID NO: 276 - protein, 15 aa, Homo sapiens
CVVTEASGGSYIPTF

SEQ ID NO: 277 - protein, 15 aa, Homo sapiens
CVVTGAAGGSYIPTF

SEQ ID NO: 278 - protein, 15 aa, Homo sapiens
CVVTIAEGGSYIPTF

SEQ ID NO: 279 - protein, 15 aa, Homo sapiens
CVVTNAPGGSYIPTF

SEQ ID NO: 280 - protein, 15 aa, Homo sapiens
CVVTPAPGGSYIPTF

SEQ ID NO: 281 - protein, 15 aa, Homo sapiens
CVVTRASGGSYIPTF

SEQ ID NO: 282 - protein, 15 aa, Homo sapiens
CVVTSARGGSYIPTF

SEQ ID NO: 283 - protein, 15 aa, Homo sapiens
CVVTSATGGSYIPTF

SEQ ID NO: 284 - protein, 15 aa, Homo sapiens
CVVTTAGGGSYIPTF

SEQ ID NO: 285 - protein, 15 aa, Homo sapiens
CVVVFASGGSYIPTF

SEQ ID NO: 286 - protein, 15 aa, Homo sapiens
CVVVGASGGSYIPTF

SEQ ID NO: 287 - protein, 15 aa, Homo sapiens
CVVVMASGGSYIPTF

SEQ ID NO: 288 - protein, 15 aa, Homo sapiens
CVVVRASGGSYIPTF

SEQ ID NO: 289 - protein, 15 aa, Homo sapiens
CVVWGASGGSYIPTF

SEQ ID NO: 290 - protein, 15 aa, Homo sapiens
CVVWPASGGSYIPTF

SEQ ID NO: 291 - protein, 15 aa, Homo sapiens
CVVWTASGGSYIPTF

SEQ ID NO: 292 - protein, 15 aa, Homo sapiens
CVVYFASGGSYIPTF

SEQ ID NO: 293 - protein, 15 aa, Homo sapiens
CVVYGASGGSYIPTF

SEQ ID NO: 294 - protein, 15 aa, Homo sapiens
CVVYMAPGGSYIPTF

SEQ ID NO: 295 - protein, 15 aa, Homo sapiens
CVVYPASGGSYIPTF

SEQ ID NO: 296 - DNA, 45 bp, Homo sapiens
tgtgtggtgaacattgcatcaggaggaagctacatacctacattt

SEQ ID NO: 297 - DNA, 45 bp, Homo sapiens
tgtgtggtgaacttggcatcaggaggaagctacatacctacattt

SEQ ID NO: 298 - DNA, 45 bp, Homo sapiens
tgtgtggtgaacaaggcggcaggaggaagctacatacctacattt

SEQ ID NO: 299 - DNA, 45 bp, Homo sapiens
tgtgtggtccgaattgcatcaggaggaagctacatacctacattt

SEQ ID NO: 300 - DNA, 45 bp, Homo sapiens
tgtgtggtgattcatgcatcaggaggaagctacatacctacattt

SEQ ID NO: 301 - DNA, 45 bp, Homo sapiens
tgtgtggtgaggggagcatcaggaggaagctacatacctacattt

SEQ ID NO: 302 - DNA, 45 bp, Homo sapiens
tgtgtggtgagaaaggcgtcaggaggaagctacatacctacattt

SEQ ID NO: 303 - DNA, 45 bp, Homo sapiens
tgtgtggtgaacttcgcatcaggaggaagctacatacctacattt

SEQ ID NO: 304 - DNA, 45 bp, Homo sapiens
tgtgtggtgaaccttgcatcaggaggaagctacatacctacattt

SEQ ID NO: 305 - DNA, 45 bp, Homo sapiens
tgtgtggtgaacctcgcatcaggaggaagctacatacctacattt

SEQ ID NO: 306 - DNA, 45 bp, Homo sapiens
tgtgtggtgaacacggcatcaggaggaagctacatacctacattt

SEQ ID NO: 307 - DNA, 45 bp, Homo sapiens
tgtgtggtgaacagagccccaggaggaagctacatacctacattt

SEQ ID NO: 308 - DNA, 45 bp, Homo sapiens
tgtgtggtgagggtggcatcaggaggaagctacatacctacattt

SEQ ID NO: 309 - DNA, 45 bp, Homo sapiens
tgtgtggtccgtttcgcatcaggaggaagctacatacctacattt

SEQ ID NO: 310 - DNA, 45 bp, Homo sapiens
tgtgtggtgaccgtagcatcaggaggaagctacatacctacattt

SEQ ID NO: 311 - DNA, 45 bp, Homo sapiens
tgtgtggtgaacgccgcatcaggaggaagctacatacctacattt

SEQ ID NO: 312 - DNA, 45 bp, Homo sapiens
tgtgtggtgaacatcgcatcaggaggaagctacatacctacattt

SEQ ID NO: 313 - DNA, 45 bp, Homo sapiens
tgtgtggtgaacggcgcatcaggaggaagctacatacctacattt

SEQ ID NO: 314 - DNA, 45 bp, Homo sapiens
tgtgtggtgagccttgcatcaggaggaagctacatacctacattt

SEQ ID NO: 315 - DNA, 45 bp, Homo sapiens
tgtgtggttcgttttgcatcaggaggaagctacatacctacattt

SEQ ID NO: 316 - DNA, 45 bp, Homo sapiens
tgtgtggtgaggtttgcatcaggaggaagctacatacctacattt

SEQ ID NO: 317 - DNA, 45 bp, Homo sapiens
tgtgtggtgcgttcggcatcaggaggaagctacatacctacattt

SEQ ID NO: 318 - DNA, 45 bp, Homo sapiens
tgtgtggtgagcttagcatcaggaggaagctacatacctacattt

SEQ ID NO: 319 - DNA, 45 bp, Homo sapiens
tgtgtggttaaacttgcatcaggaggaagctacatacctacattt

SEQ ID NO: 320 - DNA, 45 bp, Homo sapiens
tgtgtggtgaactttgcatcaggaggaagctacatacctacattt

SEQ ID NO: 321 - DNA, 45 bp, Homo sapiens
tgtgtggtgaggctcgcatcaggaggaagctacatacctacattt

SEQ ID NO: 322 - DNA, 45 bp, Homo sapiens
tgtgtggtgagggtcgcatcaggaggaagctacatacctacattt

SEQ ID NO: 323 - DNA, 45 bp, Homo sapiens
tgtgtggtgaggcatgcatcaggaggaagctacatacctacattt

SEQ ID NO: 324 - DNA, 45 bp, Homo sapiens
tgtgtggtgaggaccgcatcaggaggaagctacatacctacattt

SEQ ID NO: 325 - DNA, 45 bp, Homo sapiens
tgtgtggtgagagccgcatcaggaggaagctacatacctacattt

SEQ ID NO: 326 - DNA, 45 bp, Homo sapiens
tgtgtggtgaacaccgcatcaggaggaagctacatacctacattt

SEQ ID NO: 327 - DNA, 45 bp, Homo sapiens
tgtgtggtccgacgggcatcaggaggaagctacatacctacattt

SEQ ID NO: 328 - DNA, 45 bp, Homo sapiens
tgtgtggtgactttagcatcaggaggaagctacatacctacattt

SEQ ID NO: 329 - DNA, 45 bp, Homo sapiens
tgtgtggtgacgttcgcatcaggaggaagctacatacctacattt

SEQ ID NO: 330 - DNA, 45 bp, Homo sapiens
tgtgtggtgagcgtggcatcaggaggaagctacatacctacattt

SEQ ID NO: 331 - DNA, 45 bp, Homo sapiens
tgtgtggtgaggggggcatcaggaggaagctacatacctacattt

SEQ ID NO: 332 - DNA, 45 bp, Homo sapiens
tgtgtggtgaggacggcatcaggaggaagctacatacctacattt

SEQ ID NO: 333 - DNA, 45 bp, Homo sapiens
tgtgtggtgaactctgcatcaggaggaagctacatacctacattt

SEQ ID NO: 334 - DNA, 45 bp, Homo sapiens
tgtgtggtgaactcggctggaggaggaagctacatacctacattt

SEQ ID NO: 335 - DNA, 45 bp, Homo sapiens
tgtgtggtgaaccttgcctcaggaggaagctacatacctacattt

SEQ ID NO: 336 - DNA, 45 bp, Homo sapiens
tgtgtggtgaacatggcatcaggaggaagctacatacctacattt

SEQ ID NO: 337 - DNA, 45 bp, Homo sapiens
tgtgtggtgaacagggcatcaggaggaagctacatacctacattt

SEQ ID NO: 338 - DNA, 45 bp, Homo sapiens
tgtgtggtgaacacagcggcaggaggaagctacatacctacattt

SEQ ID NO: 339 - DNA, 45 bp, Homo sapiens
tgtgtggtgaatcttgcatcaggaggaagctacatacctacattt

SEQ ID NO: 340 - DNA, 45 bp, Homo sapiens
tgtgtggtgaccgtcgcatcaggaggaagctacatacctacattt

SEQ ID NO: 341 - DNA, 45 bp, Homo sapiens
tgtgtggtgaggagcgccacaggaggaagctacatacctacattt

SEQ ID NO: 342 - DNA, 45 bp, Homo sapiens
tgtgtggtgaacgtagcatcaggaggaagctacatacctacattt

SEQ ID NO: 343 - DNA, 45 bp, Homo sapiens
tgtgtggtgaacatagcatcaggaggaagctacatacctacattt

SEQ ID NO: 344 - DNA, 45 bp, Homo sapiens
tgtgtggtccgccaggcatcaggaggaagctacatacctacattt

SEQ ID NO: 345 - DNA, 45 bp, Homo sapiens
tgtgtggtgacctttgcatcaggaggaagctacatacctacattt

SEQ ID NO: 346 - DNA, 45 bp, Homo sapiens
tgtgtggtgagcctggcaaagggaggaagctacatacctacattt

SEQ ID NO: 347 - DNA, 45 bp, Homo sapiens
tgtgtggtgagcaccgcttcaggaggaagctacatacctacattt

SEQ ID NO: 348 - DNA, 45 bp, Homo sapiens
tgtgtggtgaggcgtgcatcaggaggaagctacatacctacattt

SEQ ID NO: 349 - DNA, 45 bp, Homo sapiens
tgtgtggtgaggagtgcatcaggaggaagctacatacctacattt

SEQ ID NO: 350 - DNA, 45 bp, Homo sapiens
tgtgtggtgaacctggcggggggaggaagctacatacctacattt

SEQ ID NO: 351 - DNA, 45 bp, Homo sapiens
tgtgtggtgaacggcgccgcaggaggaagctacatacctacattt

SEQ ID NO: 352 - DNA, 45 bp, Homo sapiens
tgtgtggtgaaccgggcatcaggaggaagctacatacctacattt

SEQ ID NO: 353 - DNA, 45 bp, Homo sapiens
tgtgtggtgaacatggcgggaggaggaagctacatacctacattt

SEQ ID NO: 354 - DNA, 45 bp, Homo sapiens
tgtgtggtgaccctggcatcaggaggaagctacatacctacattt

SEQ ID NO: 355 - DNA, 45 bp, Homo sapiens
tgtgtggtccgagttgcatcaggaggaagctacatacctacattt

SEQ ID NO: 356 - DNA, 45 bp, Homo sapiens
tgtgtggtgaccaccgcatcaggaggaagctacatacctacattt

SEQ ID NO: 357 - DNA, 45 bp, Homo sapiens
tgtgtggtgagcttcgcatcaggaggaagctacatacctacattt

SEQ ID NO: 358 - DNA, 45 bp, Homo sapiens
tgtgtggtgggcctagcatcaggaggaagctacatacctacattt

SEQ ID NO: 359 - DNA, 45 bp, Homo sapiens
tgtgtggtggggatagcatcaggaggaagctacatacctacattt

SEQ ID NO: 360 - DNA, 45 bp, Homo sapiens
tgtgtggtgaatctcgcatcaggaggaagctacatacctacattt

SEQ ID NO: 361 - DNA, 45 bp, Homo sapiens
tgtgtggtgaacctggcatcaggaggaagctacatacctacattt

SEQ ID NO: 362 - DNA, 45 bp, Homo sapiens
tgtgtggtgaacagtgcatcaggaggaagctacatacctacattt

SEQ ID NO: 363 - DNA, 45 bp, Homo sapiens
tgtgtggtacggtcggcatcaggaggaagctacatacctacattt

SEQ ID NO: 364 - DNA, 45 bp, Homo sapiens
tgtgtggtctcgtctgcatcaggaggaagctacatacctacattt

SEQ ID NO: 365 - DNA, 45 bp, Homo sapiens
tgtgtggtgcgtctggcatcaggaggaagctacatacctacattt

SEQ ID NO: 366 - DNA, 45 bp, Homo sapiens
tgtgtggtgcgtaccgcatcaggaggaagctacatacctacattt

SEQ ID NO: 367 - DNA, 45 bp, Homo sapiens
tgtgtggtgacggtcgcatcaggaggaagctacatacctacattt

SEQ ID NO: 368 - DNA, 45 bp, Homo sapiens
tgtgtggtgaggtccgcatcaggaggaagctacatacctacattt

SEQ ID NO: 369 - DNA, 45 bp, Homo sapiens
tgtgtggtgaggctagcatcaggaggaagctacatacctacattt

SEQ ID NO: 370 - DNA, 45 bp, Homo sapiens
tgtgtggtgaacatggcgacaggaggaagctacatacctacattt

SEQ ID NO: 371 - DNA, 45 bp, Homo sapiens
tgtgtggtgtccgaggcctcaggaggaagctacatacctacattt

SEQ ID NO: 372 - DNA, 45 bp, Homo sapiens
tgtgtggtgtcgatcgcatcaggaggaagctacatacctacattt

SEQ ID NO: 373 - DNA, 45 bp, Homo sapiens
tgtgtggtgactctcgcatcaggaggaagctacatacctacattt

SEQ ID NO: 374 - DNA, 45 bp, Homo sapiens
tgtgtggtgacccttgcatcaggaggaagctacatacctacattt

SEQ ID NO: 375 - DNA, 45 bp, Homo sapiens
tgtgtggtgaccctggcggggggaggaagctacatacctacattt

SEQ ID NO: 376 - DNA, 45 bp, Homo sapiens
tgtgtggtgacgctagcatcaggaggaagctacatacctacattt

SEQ ID NO: 377 - DNA, 45 bp, Homo sapiens
tgtgtggtgagcccagcatcaggaggaagctacatacctacattt

SEQ ID NO: 378 - DNA, 45 bp, Homo sapiens
tgtgtggtgaggttagcatcaggaggaagctacatacctacattt

SEQ ID NO: 379 - DNA, 45 bp, Homo sapiens
tgtgtggtgaggctggcatcaggaggaagctacatacctacattt

SEQ ID NO: 380 - DNA, 45 bp, Homo sapiens
tgtgtggtgagggttgcatcaggaggaagctacatacctacattt

SEQ ID NO: 381 - DNA, 45 bp, Homo sapiens
tgtgtggtgaggatcgcatcaggaggaagctacatacctacattt

SEQ ID NO: 382 - DNA, 45 bp, Homo sapiens
tgtgtggtgagacatgcatcaggaggaagctacatacctacattt

SEQ ID NO: 383 - DNA, 45 bp, Homo sapiens
tgtgtggtgaatgttgcatcaggaggaagctacatacctacattt

SEQ ID NO: 384 - DNA, 45 bp, Homo sapiens
tgtgtggtgaactctgccgcaggaggaagctacatacctacattt

SEQ ID NO: 385 - DNA, 45 bp, Homo sapiens
tgtgtggtgaacgttgcatcaggaggaagctacatacctacattt

SEQ ID NO: 386 - DNA, 45 bp, Homo sapiens
tgtgtggtgaaaacggcgggaggaggaagctacatacctacattt

SEQ ID NO: 387 - DNA, 45 bp, Homo sapiens
tgtgtggtgtaccatgcatcaggaggaagctacatacctacattt

SEQ ID NO: 388 - DNA, 45 bp, Homo sapiens
tgtgtggtgaacggagcatcaggaggaagctacatacctacattt

SEQ ID NO: 389 - DNA, 45 bp, Homo sapiens
tgtgtggtgaggcttgcatcaggaggaagctacatacctacattt

SEQ ID NO: 390 - DNA, 45 bp, Homo sapiens
tgtgtggtgaccccagcatcaggaggaagctacatacctacattt

SEQ ID NO: 391 - DNA, 45 bp, Homo sapiens
tgtgtggtgaacatagcaggaggaggaagctacatacctacattt

SEQ ID NO: 392 - DNA, 45 bp, Homo sapiens
tgtgtggtgaaccatgcatcaggaggaagctacatacctacattt

SEQ ID NO: 393 - DNA, 45 bp, Homo sapiens
tgtgtggtgaaatcggcggggggaggaagctacatacctacattt

SEQ ID NO: 394 - DNA, 45 bp, Homo sapiens
tgtgtggtgaatctagcatcaggaggaagctacatacctacattt

SEQ ID NO: 395 - DNA, 45 bp, Homo sapiens
tgtgtggtcaaaagcgcatcaggaggaagctacatacctacattt

SEQ ID NO: 396 - DNA, 45 bp, Homo sapiens
tgtgtggtgaacggggcatcaggaggaagctacatacctacattt

SEQ ID NO: 397 - DNA, 45 bp, Homo sapiens
tgtgtggtgtcgttcgcatcaggaggaagctacatacctacattt

SEQ ID NO: 398 - DNA, 45 bp, Homo sapiens
tgtgtggtgaactccgcatcaggaggaagctacatacctacattt

SEQ ID NO: 399 - DNA, 45 bp, Homo sapiens
tgtgtggttaggcatgcatcaggaggaagctacatacctacattt

SEQ ID NO: 400 - DNA, 45 bp, Homo sapiens
tgtgtggtgagggccgcatcaggaggaagctacatacctacattt

SEQ ID NO: 401 - DNA, 45 bp, Homo sapiens
tgtgtggtgaccctcgcatcaggaggaagctacatacctacattt

SEQ ID NO: 402 - DNA, 45 bp, Homo sapiens
tgtgtggtgagactagcatcaggaggaagctacatacctacattt

SEQ ID NO: 403 - DNA, 45 bp, Homo sapiens
tgtgtggtgaacggggcgtcaggaggaagctacatacctacattt

SEQ ID NO: 404 - DNA, 45 bp, Homo sapiens
tgtgtggtgaacatggcggcaggaggaagctacatacctacattt

SEQ ID NO: 405 - DNA, 45 bp, Homo sapiens
tgtgtggtgaaccaggcggcaggaggaagctacatacctacattt

SEQ ID NO: 406 - DNA, 45 bp, Homo sapiens
tgtgtggtaccccgtgcatcaggaggaagctacatacctacattt

SEQ ID NO: 407 - DNA, 45 bp, Homo sapiens
tgtgtggtgaacatagcaacaggaggaagctacatacctacattt

SEQ ID NO: 408 - DNA, 45 bp, Homo sapiens
tgtgtggttagacatgcatcaggaggaagctacatacctacattt

SEQ ID NO: 409 - DNA, 45 bp, Homo sapiens
tgtgtggtgagcctagcatcaggaggaagctacatacctacattt

SEQ ID NO: 410 - DNA, 45 bp, Homo sapiens
tgtgtggtgagagcggcatcaggaggaagctacatacctacattt

SEQ ID NO: 411 - DNA, 45 bp, Homo sapiens
tgtgtggtgaacctagcatcaggaggaagctacatacctacattt

SEQ ID NO: 412 - DNA, 45 bp, Homo sapiens
tgtgtggtgaacgtcgcatcaggaggaagctacatacctacattt

SEQ ID NO: 413 - DNA, 45 bp, Homo sapiens
tgtgtggtgagcctcgcatcaggaggaagctacatacctacattt

SEQ ID NO: 414 - DNA, 45 bp, Homo sapiens
tgtgtggtgaatacggccgggggaggaagctacatacctacattt

SEQ ID NO: 415 - DNA, 45 bp, Homo sapiens
tgtgtggtgaacatcgcggcaggaggaagctacatacctacattt

SEQ ID NO: 416 - DNA, 45 bp, Homo sapiens
tgtgtggtccttacggcatcaggaggaagctacatacctacattt

SEQ ID NO: 417 - DNA, 45 bp, Homo sapiens
tgtgtggtgtcccatgcatcaggaggaagctacatacctacattt

SEQ ID NO: 418 - DNA, 45 bp, Homo sapiens
tgtgtggtgctatccgcatcaggaggaagctacatacctacattt

SEQ ID NO: 419 - DNA, 45 bp, Homo sapiens
tgtgtggtgaccctagcatcaggaggaagctacatacctacattt

SEQ ID NO: 420 - DNA, 45 bp, Homo sapiens
tgtgtggtgagtcttgcatcaggaggaagctacatacctacattt

SEQ ID NO: 421 - DNA, 45 bp, Homo sapiens
tgtgtggtgagtggggccgtgggaggaagttacatacctacattt

SEQ ID NO: 422 - DNA, 45 bp, Homo sapiens
tgtgtggtgagtggggccgtgggaggaagctacatacctacattt

SEQ ID NO: 423 - DNA, 45 bp, Homo sapiens
tgtgtggtgagccatgcatcaggaggaagctacatacctacattt

SEQ ID NO: 424 - DNA, 45 bp, Homo sapiens
tgtgtggtgaattcagcatcaggaggaagctacatacctacattt

SEQ ID NO: 425 - DNA, 45 bp, Homo sapiens
tgtgtggtgaacatcgccgggggaggaagctacatacctacattt

SEQ ID NO: 426 - DNA, 45 bp, Homo sapiens
tgtgtggtgaacatggcttcaggaggaagctacatacctacattt

SEQ ID NO: 427 - DNA, 45 bp, Homo sapiens
tgtgtggtgaacatggcagcaggaggaagctacatacctacattt

SEQ ID NO: 428 - DNA, 45 bp, Homo sapiens
tgtgtggtgacctctgcatcaggaggaagctacatacctacattt

SEQ ID NO: 429 - DNA, 45 bp, Homo sapiens
tgtgtggtgaacttagccagaggaggaagctacatacctacattt

SEQ ID NO: 430 - DNA, 45 bp, Homo sapiens
tgtgtggtgaaccccgcatcaggaggaagctacatacctacattt

SEQ ID NO: 431 - DNA, 45 bp, Homo sapiens
tgtgtggtgaacattgcctcaggaggaagctacatacctacattt

SEQ ID NO: 432 - DNA, 45 bp, Homo sapiens
tgtgtggtgaactcagcttcaggaggaagctacatacctacattt

SEQ ID NO: 433 - DNA, 45 bp, Homo sapiens
tgtgtggtcagccaagcttcaggaggaagctacatacctacattt

SEQ ID NO: 434 - DNA, 45 bp, Homo sapiens
tgtgtggtgaacgaggcatcaggaggaagctacatacctacattt

SEQ ID NO: 435 - DNA, 45 bp, Homo sapiens
tgtgtggtgagtcatgcatcaggaggaagctacatacctacattt

SEQ ID NO: 436 - DNA, 45 bp, Homo sapiens
tgtgtggtgagcacggcaacaggaggaagctacatacctacattt

SEQ ID NO: 437 - DNA, 45 bp, Homo sapiens
tgtgtggtgaacagcgcatcaggaggaagctacatacctacattt

SEQ ID NO: 438 - DNA, 45 bp, Homo sapiens
tgtgtggtgaacagagcatcaggaggaagctacatacctacattt

SEQ ID NO: 439 - DNA, 45 bp, Homo sapiens
tgtgtggtgtatcatgcatcaggaggaagctacatacctacattt

SEQ ID NO: 440 - DNA, 45 bp, Homo sapiens
tgtgtggtgatccaagcatcaggaggaagctacatacctacattt

SEQ ID NO: 441 - DNA, 45 bp, Homo sapiens
tgtgtggtgatcgatgcatcaggaggaagctacatacctacattt

SEQ ID NO: 442 - DNA, 45 bp, Homo sapiens
tgtgtggtgaacccagcatcaggaggaagctacatacctacattt

SEQ ID NO: 443 - DNA, 45 bp, Homo sapiens
tgtgtggtgaacgaagcatcaggaggaagctacatacctacattt

SEQ ID NO: 444 - DNA, 45 bp, Homo sapiens
tgtgtggtgaacatggcgctcggaggaagctacatacctacattt

SEQ ID NO: 445 - DNA, 45 bp, Homo sapiens
tgtgtggtgatcccggcatcaggaggaagctacatacctacattt

SEQ ID NO: 446 - DNA, 45 bp, Homo sapiens
tgtgtggtgacccctgcatcaggaggaagctacatacctacattt

SEQ ID NO: 447 - DNA, 45 bp, Homo sapiens
tgtgtggtgccccgagcctcaggaggaagctacatacctacattt

SEQ ID NO: 448 - DNA, 45 bp, Homo sapiens
tgtgtggtttctcatgcatcaggaggaagctacatacctacattt

SEQ ID NO: 449 - DNA, 45 bp, Homo sapiens
tgtgtggtgtccccggccccaggaggaagctacatacctacattt

SEQ ID NO: 450 - DNA, 45 bp, Homo sapiens
tgtgtggtgaacgacgcatcaggaggaagctacatacctacattt

SEQ ID NO: 451 - DNA, 45 bp, Homo sapiens
tgtgtggtgaggaaagcatcaggaggaagctacatacctacattt

SEQ ID NO: 452 - DNA, 45 bp, Homo sapiens
tgtgtggtgaacactgcatcaggaggaagctacatacctacattt

SEQ ID NO: 453 - DNA, 45 bp, Homo sapiens
tgtgtggtccgacatgcatcaggaggaagctacatacctacattt

SEQ ID NO: 454 - DNA, 45 bp, Homo sapiens
tgtgtggtgacccccgcatcaggaggaagctacatacctacattt

SEQ ID NO: 455 - DNA, 45 bp, Homo sapiens
tgtgtggtgagtattgcatcaggaggaagctacatacctacattt

SEQ ID NO: 456 - DNA, 45 bp, Homo sapiens
tgtgtggtgagcgttgcatcaggaggaagctacatacctacattt

SEQ ID NO: 457 - DNA, 45 bp, Homo sapiens
tgtgtggtgaacgcggcgacaggaggaagctacatacctacattt

SEQ ID NO: 458 - DNA, 45 bp, Homo sapiens
tgtgtggtgaacactgccccaggaggaagctacatacctacattt

SEQ ID NO: 459 - DNA, 45 bp, Homo sapiens
tgtgtggtgaagaaggcatcaggaggaagctacatacctacattt

SEQ ID NO: 460 - DNA, 45 bp, Homo sapiens
tgtgtggttcatcatgcatcaggaggaagctacatacctacattt

SEQ ID NO: 461 - DNA, 45 bp, Homo sapiens
tgtgtggtgagggaagcatcaggaggaagctacatacctacattt

SEQ ID NO: 462 - DNA, 45 bp, Homo sapiens
tgtgtggtgatccctgcatcaggaggaagctacatacctacattt

SEQ ID NO: 463 - DNA, 45 bp, Homo sapiens
tgtgtggttgtgatggcctccggaggaagctacatacctacattt

SEQ ID NO: 464 - DNA, 45 bp, Homo sapiens
tgtgtggtgaacgctgcatcaggaggaagctacatacctacattt

SEQ ID NO: 465 - DNA, 45 bp, Homo sapiens
tgtgtggtgaaccctgcatcaggaggaagctacatacctacattt

SEQ ID NO: 466 - DNA, 45 bp, Homo sapiens
tgtgtggtgaacaaagcatcaggaggaagctacatacctacattt

SEQ ID NO: 467 - DNA, 45 bp, Homo sapiens
tgtgtggtgaacatggcctcaggaggaagctacatacctacattt

SEQ ID NO: 468 - DNA, 45 bp, Homo sapiens
tgtgtggtgaacatcgcgctaggaggaagctacatacctacattt

SEQ ID NO: 469 - DNA, 45 bp, Homo sapiens
tgtgtggtgaacgtagcaacaggaggaagctacatacctacattt

SEQ ID NO: 470 - DNA, 45 bp, Homo sapiens
tgtgtggtgcaccaggcatcaggaggaagctacatacctacattt

SEQ ID NO: 471 - DNA, 45 bp, Homo sapiens
tgtgtggtgaacctggctgggggaggaagctacatacctacattt

SEQ ID NO: 472 - DNA, 45 bp, Homo sapiens
tgtgtggttcgacatgcatcaggaggaagctacatacctacattt

SEQ ID NO: 473 - DNA, 45 bp, Homo sapiens
tgtgtggtgaaccgtgcatcaggaggaagctacatacctacattt

SEQ ID NO: 474 - DNA, 45 bp, Homo sapiens
tgtgtggtccaccatgcatcaggaggaagctacatacctacattt

SEQ ID NO: 475 - DNA, 45 bp, Homo sapiens
tgtgtggtgagaactgcatcaggaggaagctacatacctacattt

SEQ ID NO: 476 - DNA, 45 bp, Homo sapiens
tgtgtggtgaactcggcatcaggaggaagctacatacctacattt

SEQ ID NO: 477 - DNA, 45 bp, Homo sapiens
tgtgtggttcgtcttgcatcaggaggaagctacatacctacattt

SEQ ID NO: 478 - DNA, 45 bp, Homo sapiens
tgtgtggttagccatgcatcaggaggaagctacatacctacattt

SEQ ID NO: 479 - DNA, 45 bp, Homo sapiens
tgtgtggtgtcacatgcatcaggaggaagctacatacctacattt

SEQ ID NO: 480 - DNA, 45 bp, Homo sapiens
tgtgtggtgctcaccgcatcaggaggaagctacatacctacattt

SEQ ID NO: 481 - DNA, 45 bp, Homo sapiens
tgtgtggtgccccatgcatcaggaggaagctacatacctacattt

SEQ ID NO: 482 - DNA, 45 bp, Homo sapiens
tgtgtggtgatcgcggcatcaggaggaagctacatacctacattt

SEQ ID NO: 483 - DNA, 45 bp, Homo sapiens
tgtgtggtgagggtagcggcaggaggaagctacatacctacattt

SEQ ID NO: 484 - DNA, 45 bp, Homo sapiens
tgtgtggtgagagaggcatcaggaggaagctacatacctacattt

SEQ ID NO: 485 - DNA, 45 bp, Homo sapiens
tgtgtggtgaaatccgcatcaggaggaagctacatacctacattt

SEQ ID NO: 486 - DNA, 45 bp, Homo sapiens
tgtgtggtgaattctgcatcaggaggaagctacatacctacattt

SEQ ID NO: 487 - DNA, 45 bp, Homo sapiens
tgtgtggtgaacccggcatcaggaggaagctacatacctacattt

SEQ ID NO: 488 - DNA, 45 bp, Homo sapiens
tgtgtggtgcttagcgcatcaggaggaagctacatacctacattt

SEQ ID NO: 489 - DNA, 45 bp, Homo sapiens
tgtgtggtgagcgccgcatcaggaggaagctacatacctacattt

SEQ ID NO: 490 - DNA, 45 bp, Homo sapiens
tgtgtggtgaacatagctgcaggaggaagctacatacctacattt

SEQ ID NO: 491 - DNA, 45 bp, Homo sapiens
tgtgtggtgggggtcgcatcaggaggaagctacatacctacattt

SEQ ID NO: 492 - DNA, 45 bp, Homo sapiens
tgtgtggtgagcaccgcatcaggaggaagctacatacctacattt

SEQ ID NO: 493 - DNA, 45 bp, Homo sapiens
tgtgtggtgcgtcatgcatcaggaggaagctacatacctacattt

SEQ ID NO: 494 - DNA, 45 bp, Homo sapiens
tgtgtggtgaccattgcggagggaggaagctacatacctacattt

SEQ ID NO: 495 - DNA, 45 bp, Homo sapiens
tgtgtggtgagcgcggcatcaggaggaagctacatacctacattt

SEQ ID NO: 496 - DNA, 45 bp, Homo sapiens
tgtgtggtgaggattgcatcaggaggaagctacatacctacattt

SEQ ID NO: 497 - DNA, 45 bp, Homo sapiens
tgtgtggtgaaccgggcaacaggaggaagctacatacctacattt

SEQ ID NO: 498 - DNA, 45 bp, Homo sapiens
tgtgtggtgaacgaggcggcaggaggaagctacatacctacattt

SEQ ID NO: 499 - DNA, 45 bp, Homo sapiens
tgtgtggtgaacatagcggcaggaggaagctacatacctacattt

SEQ ID NO: 500 - DNA, 45 bp, Homo sapiens
tgtgtggtgaacacggctaaaggaggaagctacatacctacattt

SEQ ID NO: 501 - DNA, 45 bp, Homo sapiens
tgtgtggtgagtgcggcatcaggaggaagctacatacctacattt

SEQ ID NO: 502 - DNA, 45 bp, Homo sapiens
tgtgtggttcgtcatgcatcaggaggaagctacatacctacattt

SEQ ID NO: 503 - DNA, 45 bp, Homo sapiens
tgtgtggtgtcttttgcatcaggaggaagctacatacctacattt

SEQ ID NO: 504 - DNA, 45 bp, Homo sapiens
tgtgtggtgaccattgcatcaggaggaagctacatacctacattt

SEQ ID NO: 505 - DNA, 45 bp, Homo sapiens
tgtgtggtgaggggcgcatcaggaggaagctacatacctacattt

SEQ ID NO: 506 - DNA, 45 bp, Homo sapiens
tgtgtggtgaacgtcgcgtcaggaggaagctacatacctacattt

SEQ ID NO: 507 - DNA, 45 bp, Homo sapiens
tgtgtggtgaagggagcatcaggaggaagctacatacctacattt

SEQ ID NO: 508 - DNA, 45 bp, Homo sapiens
tgtgtggtgaacggcgcgccaggaggaagctacatacctacattt

SEQ ID NO: 509 - DNA, 45 bp, Homo sapiens
tgtgtggtgttccgagcatcaggaggaagctacatacctacattt

SEQ ID NO: 510 - DNA, 45 bp, Homo sapiens
tgtgtggtgtctcttgcatcaggaggaagctacatacctacattt

SEQ ID NO: 511 - DNA, 45 bp, Homo sapiens
tgtgtggtgacgctcgcatcaggaggaagctacatacctacattt

SEQ ID NO: 512 - DNA, 45 bp, Homo sapiens
tgtgtggtgaacatagcagcaggaggaagctacatacctacattt

SEQ ID NO: 513 - DNA, 45 bp, Homo sapiens
tgtgtggtctctatagcatcaggaggaagctacatacctacattt

SEQ ID NO: 514 - DNA, 45 bp, Homo sapiens
tgtgtggtgttccatgcatcaggaggaagctacatacctacattt

SEQ ID NO: 515 - DNA, 45 bp, Homo sapiens
tgtgtggtgaagagggctggaggaggaagctacatacctacattt

SEQ ID NO: 516 - DNA, 45 bp, Homo sapiens
tgtgtggtgagccgcgcatcaggaggaagctacatacctacattt

SEQ ID NO: 517 - DNA, 45 bp, Homo sapiens
tgtgtggtgaacatcgcgacaggaggaagctacatacctacattt

SEQ ID NO: 518 - DNA, 45 bp, Homo sapiens
tgtgtggtgatccccgcatcaggaggaagctacatacctacattt

SEQ ID NO: 519 - DNA, 45 bp, Homo sapiens
tgtgtggtgaactcagcatcaggaggaagctacatacctacattt

SEQ ID NO: 520 - DNA, 45 bp, Homo sapiens
tgtgtggtgaactacgcatcaggaggaagctacatacctacattt

SEQ ID NO: 521 - DNA, 45 bp, Homo sapiens
tgtgtggtgaacggggcgacaggaggaagctacatacctacattt

SEQ ID NO: 522 - DNA, 45 bp, Homo sapiens
tgtgtggtgaacaaggcatcaggaggaagctacatacctacattt

SEQ ID NO: 523 - DNA, 45 bp, Homo sapiens
tgtgtggtgaagcatgcatcaggaggaagctacatacctacattt

SEQ ID NO: 524 - DNA, 45 bp, Homo sapiens
tgtgtggtgaaacccgcatcaggaggaagctacatacctacattt

SEQ ID NO: 525 - DNA, 45 bp, Homo sapiens
tgtgtggtgatttccgcatcaggaggaagctacatacctacattt

SEQ ID NO: 526 - DNA, 45 bp, Homo sapiens
tgtgtggtgatccgtgcatcaggaggaagctacatacctacattt

SEQ ID NO: 527 - DNA, 45 bp, Homo sapiens
tgtgtggtgaccgctgcatcaggaggaagctacatacctacattt

SEQ ID NO: 528 - DNA, 45 bp, Homo sapiens
tgtgtggtgaaaggggcatcaggaggaagctacatacctacattt

SEQ ID NO: 529 - DNA, 45 bp, Homo sapiens
tgtgtggtcttccttgcatcaggaggaagctacatacctacattt

SEQ ID NO: 530 - DNA, 45 bp, Homo sapiens
tgtgtggtgaaccaagcatcaggaggaagctacatacctacattt

SEQ ID NO: 531 - DNA, 45 bp, Homo sapiens
tgtgtggtgaacattgcaacaggaggaagctacatacctacattt

SEQ ID NO: 532 - DNA, 45 bp, Homo sapiens
tgtgtggtgtccttagcatcaggaggaagctacatacctacattt

SEQ ID NO: 533 - DNA, 45 bp, Homo sapiens
tgtgtggtgcggcttgcatcaggaggaagctacatacctacattt

SEQ ID NO: 534 - DNA, 45 bp, Homo sapiens
tgtgtggtccgccccgcgtcaggaggaagctacatacctacattt

SEQ ID NO: 535 - DNA, 45 bp, Homo sapiens
tgtgtggtgagtgttgcatcaggaggaagctacatacctacattt

SEQ ID NO: 536 - DNA, 45 bp, Homo sapiens
tgtgtggtgttttccgcatcaggaggaagctacatacctacattt

SEQ ID NO: 537 - DNA, 45 bp, Homo sapiens
tgtgtggtgaccccggcaccaggaggaagctacatacctacattt

SEQ ID NO: 538 - DNA, 45 bp, Homo sapiens
tgtgtggtgagtaccgcatcaggaggaagctacatacctacattt

SEQ ID NO: 539 - DNA, 45 bp, Homo sapiens
tgtgtggtgattccagcatcaggaggaagctacatacctacattt

SEQ ID NO: 540 - DNA, 45 bp, Homo sapiens
tgtgtggtgaatcatgcatcaggaggaagctacatacctacattt

SEQ ID NO: 541 - DNA, 45 bp, Homo sapiens
tgtgtggtgaaccaggcatcaggaggaagctacatacctacattt

SEQ ID NO: 542 - DNA, 45 bp, Homo sapiens
tgtgtggtgaacgcggcatcaggaggaagctacatacctacattt

SEQ ID NO: 543 - DNA, 45 bp, Homo sapiens
tgtgtggtgaacggagcgtcaggaggaagctacatacctacattt

SEQ ID NO: 544 - DNA, 45 bp, Homo sapiens
tgtgtggtgaagttggcatcaggaggaagctacatacctacattt

SEQ ID NO: 545 - DNA, 45 bp, Homo sapiens
tgtgtggtggctactgcatcaggaggaagctacatacctacattt

SEQ ID NO: 546 - DNA, 45 bp, Homo sapiens
tgtgtggtgatgcccgcatcaggaggaagctacatacctacattt

SEQ ID NO: 547 - DNA, 45 bp, Homo sapiens
tgtgtggtctccttagcatcaggaggaagctacatacctacattt

SEQ ID NO: 548 - DNA, 45 bp, Homo sapiens
tgtgtggtgagggaggcatcaggaggaagctacatacctacattt

SEQ ID NO: 549 - DNA, 45 bp, Homo sapiens
tgtgtggtgaacattgcagggggaggaagctacatacctacattt

SEQ ID NO: 550 - DNA, 45 bp, Homo sapiens
tgtgtggtgcgcctcgcatcaggaggaagctacatacctacattt

SEQ ID NO: 551 - DNA, 45 bp, Homo sapiens
tgtgtggtgcgcaccgcatcaggaggaagctacatacctacattt

SEQ ID NO: 552 - DNA, 45 bp, Homo sapiens
tgtgtggtgagcattgcatcaggaggaagctacatacctacattt

SEQ ID NO: 553 - DNA, 45 bp, Homo sapiens
tgtgtggtgagacgagcatcaggaggaagctacatacctacattt

SEQ ID NO: 554 - DNA, 45 bp, Homo sapiens
tgtgtggtttctatcgcatcaggaggaagctacatacctacattt

SEQ ID NO: 555 - DNA, 45 bp, Homo sapiens
tgtgtggttaagaaggcatcaggaggaagctacatacctacattt

SEQ ID NO: 556 - DNA, 45 bp, Homo sapiens
tgtgtggtgaggttggcatcaggaggaagctacatacctacattt

SEQ ID NO: 557 - DNA, 45 bp, Homo sapiens
tgtgtggtgcgcttggcatcaggaggaagctacatacctacattt

SEQ ID NO: 558 - DNA, 45 bp, Homo sapiens
tgtgtggtgcgagaggcatcaggaggaagctacatacctacattt

SEQ ID NO: 559 - DNA, 45 bp, Homo sapiens
tgtgtggtgagtctcgcatcaggaggaagctacatacctacattt

SEQ ID NO: 560 - DNA, 45 bp, Homo sapiens
tgtgtggtctttgctgcatcaggaggaagctacatacctacattt

SEQ ID NO: 561 - DNA, 45 bp, Homo sapiens
tgtgtggtgttcctcgcggggggaggaagctacatacctacattt

SEQ ID NO: 562 - DNA, 45 bp, Homo sapiens
tgtgtggtgtccaaggcatcaggaggaagctacatacctacattt

SEQ ID NO: 563 - DNA, 45 bp, Homo sapiens
tgtgtggtgtcgcttgcatcaggaggaagctacatacctacattt

SEQ ID NO: 564 - DNA, 45 bp, Homo sapiens
tgtgtggtgagactggcttcaggaggaagctacatacctacattt

SEQ ID NO: 565 - DNA, 45 bp, Homo sapiens
tgtgtggtggctcaagcatcaggaggaagctacatacctacattt

SEQ ID NO: 566 - DNA, 45 bp, Homo sapiens
tgtgtggtgaagagggcctccggaggaagctacatacctacattt

SEQ ID NO: 567 - DNA, 45 bp, Homo sapiens
tgtgtggtgttctcggcatcaggaggaagctacatacctacattt

SEQ ID NO: 568 - DNA, 45 bp, Homo sapiens
tgtgtggtgagctccgcatcaggaggaagctacatacctacattt

SEQ ID NO: 569 - DNA, 45 bp, Homo sapiens
tgtgtggtgcctcatgcatcaggaggaagctacatacctacattt

SEQ ID NO: 570 - DNA, 45 bp, Homo sapiens
tgtgtggtgagcaaggcatcaggaggaagctacatacctacattt

SEQ ID NO: 571 - DNA, 45 bp, Homo sapiens
tgtgtggtgaacagggcgacaggaggaagctacatacctacattt

SEQ ID NO: 572 - DNA, 45 bp, Homo sapiens
tgtgtggtgaagggtgcatcaggaggaagctacatacctacattt

SEQ ID NO: 573 - DNA, 45 bp, Homo sapiens
tgtgtggtgcgccatgcatcaggaggaagctacatacctacattt

SEQ ID NO: 574 - DNA, 45 bp, Homo sapiens
tgtgtggtgaccgccgcctcaggaggaagctacatacctacattt

SEQ ID NO: 575 - DNA, 45 bp, Homo sapiens
tgtgtggtgagcgtcgcatcaggaggaagctacatacctacattt

SEQ ID NO: 576 - DNA, 45 bp, Homo sapiens
tgtgtggtgaacatggcccaaggaggaagctacatacctacattt

SEQ ID NO: 577 - DNA, 45 bp, Homo sapiens
tgtgtggtgaacatagccatcggaggaagctacatacctacattt

SEQ ID NO: 578 - DNA, 45 bp, Homo sapiens
tgtgtggtgaacatagcgtcaggaggaagctacatacctacattt

SEQ ID NO: 579 - DNA, 45 bp, Homo sapiens
tgtgtggtgtccgtcgcatcaggaggaagctacatacctacattt

SEQ ID NO: 580 - DNA, 45 bp, Homo sapiens
tgtgtggtgagttctgcatcaggaggaagctacatacctacattt

SEQ ID NO: 581 - DNA, 45 bp, Homo sapiens
tgtgtggtgtcccttgcatcaggaggaagctacatacctacattt

SEQ ID NO: 582 - DNA, 45 bp, Homo sapiens
tgtgtggtgaacaaagcctcaggaggaagctacatacctacattt

SEQ ID NO: 583 - DNA, 45 bp, Homo sapiens
tgtgtggtgatcatcgcatcaggaggaagctacatacctacattt

SEQ ID NO: 584 - DNA, 45 bp, Homo sapiens
tgtgtggtgaacggggcgccaggaggaagctacatacctacattt

SEQ ID NO: 585 - DNA, 45 bp, Homo sapiens
tgtgtggtgaaaacggcggcaggaggaagctacatacctacattt

SEQ ID NO: 586 - DNA, 45 bp, Homo sapiens
tgtgtggtccgcgtagcatcaggaggaagctacatacctacattt

SEQ ID NO: 587 - DNA, 45 bp, Homo sapiens
tgtgtggtgagatcggcatcaggaggaagctacatacctacattt

SEQ ID NO: 588 - DNA, 45 bp, Homo sapiens
tgtgtggtgaacatggcgtcaggaggaagctacatacctacattt

SEQ ID NO: 589 - DNA, 45 bp, Homo sapiens
tgtgtggtgagaatcgcatcaggaggaagctacatacctacattt

SEQ ID NO: 590 - DNA, 45 bp, Homo sapiens
tgtgtggtgaccttggcctcaggaggaagctacatacctacattt

SEQ ID NO: 591 - DNA, 45 bp, Homo sapiens
tgtgtggtggcgtcagcatcaggaggaagctacatacctacattt

SEQ ID NO: 592 - DNA, 45 bp, Homo sapiens
tgtgtggtgaacatcgcgtcaggaggaagctacatacctacattt

SEQ ID NO: 593 - DNA, 45 bp, Homo sapiens
tgtgtggtgtcgctcgcatcaggaggaagctacatacctacattt

SEQ ID NO: 594 - DNA, 45 bp, Homo sapiens
tgtgtggtgagcctggccgggggaggaagctacatacctacattt

SEQ ID NO: 595 - DNA, 45 bp, Homo sapiens
tgtgtggtgaaccgagcatcaggaggaagctacatacctacattt

SEQ ID NO: 596 - DNA, 45 bp, Homo sapiens
tgtgtggtgaatagtgcatcaggaggaagctacatacctacattt

SEQ ID NO: 597 - DNA, 45 bp, Homo sapiens
tgtgtggtgaacggcgcggcaggaggaagctacatacctacattt

SEQ ID NO: 598 - DNA, 45 bp, Homo sapiens
tgtgtggtgaacttagcatcaggaggaagctacatacctacattt

SEQ ID NO: 599 - DNA, 45 bp, Homo sapiens
tgtgtggtggccctcgcatcaggaggaagctacatacctacattt

SEQ ID NO: 600 - DNA, 45 bp, Homo sapiens
tgtgtggtcaagatcgcatcaggaggaagctacatacctacattt

SEQ ID NO: 601 - DNA, 45 bp, Homo sapiens
tgtgtggtgtcgggggcgtcaggaggaagctacatacctacattt

SEQ ID NO: 602 - DNA, 45 bp, Homo sapiens
tgtgtggtgactactgcatcaggaggaagctacatacctacattt

SEQ ID NO: 603 - DNA, 45 bp, Homo sapiens
tgtgtggtgagcacagcatcaggaggaagctacatacctacattt

SEQ ID NO: 604 - DNA, 45 bp, Homo sapiens
tgtgtggtgagacaggccgggggaggaagctacatacctacattt

SEQ ID NO: 605 - DNA, 45 bp, Homo sapiens
tgtgtggtgaacctcgcccgcggaggaagctacatacctacattt

SEQ ID NO: 606 - DNA, 45 bp, Homo sapiens
tgtgtggtgaacatggcaacaggaggaagctacatacctacattt

SEQ ID NO: 607 - DNA, 45 bp, Homo sapiens
tgtgtggtgtctcgagcatcaggaggaagctacatacctacattt

SEQ ID NO: 608 - DNA, 45 bp, Homo sapiens
tgtgtggtgaatcgtgcatcaggaggaagctacatacctacattt

SEQ ID NO: 609 - DNA, 45 bp, Homo sapiens
tgtgtggtgaacatcgcctcaggaggaagctacatacctacattt

SEQ ID NO: 610 - DNA, 45 bp, Homo sapiens
tgtgtggtttctcgagcatcaggaggaagctacatacctacattt

SEQ ID NO: 611 - DNA, 45 bp, Homo sapiens
tgtgtggtgtcgcaggcggcaggaggaagctacatacctacattt

SEQ ID NO: 612 - DNA, 45 bp, Homo sapiens
tgtgtggtgcttctagcatcaggaggaagctacatacctacattt

SEQ ID NO: 613 - DNA, 45 bp, Homo sapiens
tgtgtggtgatcgccgcatcaggaggaagctacatacctacattt

SEQ ID NO: 614 - DNA, 45 bp, Homo sapiens
tgtgtggtgaccatcgcatcaggaggaagctacatacctacattt

SEQ ID NO: 615 - DNA, 45 bp, Homo sapiens
tgtgtggtgagcccggcatcaggaggaagctacatacctacattt

SEQ ID NO: 616 - DNA, 45 bp, Homo sapiens
tgtgtggtgcggcatgcatcaggaggaagctacatacctacattt

SEQ ID NO: 617 - DNA, 45 bp, Homo sapiens
tgtgtggtgaaccgcgcatcaggaggaagctacatacctacattt

SEQ ID NO: 618 - DNA, 45 bp, Homo sapiens
tgtgtggtgaactgggcatcaggaggaagctacatacctacattt

SEQ ID NO: 619 - DNA, 45 bp, Homo sapiens
tgtgtggtgggcaccgcatcaggaggaagctacatacctacattt

SEQ ID NO: 620 - DNA, 45 bp, Homo sapiens
tgtgtggtgatcggcgcatcaggaggaagctacatacctacattt

SEQ ID NO: 621 - DNA, 45 bp, Homo sapiens
tgtgtggtccgcatggcatcaggaggaagctacatacctacattt

SEQ ID NO: 622 - DNA, 45 bp, Homo sapiens
tgtgtggtgatttttgcatcaggaggaagctacatacctacattt

SEQ ID NO: 623 - DNA, 45 bp, Homo sapiens
tgtgtggtgatctccgcatcaggaggaagctacatacctacattt

SEQ ID NO: 624 - DNA, 45 bp, Homo sapiens
tgtgtggtgacttccgcatcaggaggaagctacatacctacattt

SEQ ID NO: 625 - DNA, 45 bp, Homo sapiens
tgtgtggtgagccgagcctcaggaggaagctacatacctacattt

SEQ ID NO: 626 - DNA, 45 bp, Homo sapiens
tgtgtggtgtcgctggcatcaggaggaagctacatacctacattt

SEQ ID NO: 627 - DNA, 45 bp, Homo sapiens
tgtgtggtgaggcaggcatcaggaggaagctacatacctacattt

SEQ ID NO: 628 - DNA, 45 bp, Homo sapiens
tgtgtggtccgtctcgcatcaggaggaagctacatacctacattt

SEQ ID NO: 629 - DNA, 45 bp, Homo sapiens
tgtgtggtgagtggggcatcaggaggaagctacatacctacattt

SEQ ID NO: 630 - DNA, 45 bp, Homo sapiens
tgtgtggtgaccttcgcatcaggaggaagctacatacctacattt

SEQ ID NO: 631 - DNA, 45 bp, Homo sapiens
tgtgtggtgagggtcgcttcaggaggaagctacatacctacattt

SEQ ID NO: 632 - DNA, 45 bp, Homo sapiens
tgtgtggtgcgaacggcatcaggaggaagctacatacctacattt

SEQ ID NO: 633 - DNA, 45 bp, Homo sapiens
tgtgtggtgaagcgggcatcaggaggaagctacatacctacattt

SEQ ID NO: 634 - DNA, 45 bp, Homo sapiens
tgtgtggtcttccatgcatcaggaggaagctacatacctacattt

SEQ ID NO: 635 - DNA, 45 bp, Homo sapiens
tgtgtggtgaaggtcgcatcaggaggaagctacatacctacattt

SEQ ID NO: 636 - DNA, 45 bp, Homo sapiens
tgtgtggtggggttggcatcaggaggaagctacatacctacattt

SEQ ID NO: 637 - DNA, 45 bp, Homo sapiens
tgtgtggtgtcctcggcatcaggaggaagctacatacctacattt

SEQ ID NO: 638 - DNA, 45 bp, Homo sapiens
tgtgtggtgagctctgcatcaggaggaagctacatacctacattt

SEQ ID NO: 639 - DNA, 45 bp, Homo sapiens
tgtgtggtgaggtttgctcgaggaggaagctacatacctacattt

SEQ ID NO: 640 - DNA, 45 bp, Homo sapiens
tgtgtggtgagaacggcatcaggaggaagctacatacctacattt

SEQ ID NO: 641 - DNA, 45 bp, Homo sapiens
tgtgtggtgaattccgcatcaggaggaagctacatacctacattt

SEQ ID NO: 642 - DNA, 45 bp, Homo sapiens
tgtgtggtgaatcaagcttcaggaggaagctacatacctacattt

SEQ ID NO: 643 - DNA, 45 bp, Homo sapiens
tgtgtggtgaagatcgcatcaggaggaagctacatacctacattt

SEQ ID NO: 644 - DNA, 45 bp, Homo sapiens
tgtgtggtcctacatgcatcaggaggaagctacatacctacattt

SEQ ID NO: 645 - DNA, 45 bp, Homo sapiens
tgtgtggtgagttccgcggtaggaggaagctacatacctacattt

SEQ ID NO: 646 - DNA, 45 bp, Homo sapiens
tgtgtggtgaagttcgcatcaggaggaagctacatacctacattt

SEQ ID NO: 647 - DNA, 45 bp, Homo sapiens
tgtgtggtgagtagcgcatcaggaggaagctacatacctacattt

SEQ ID NO: 648 - DNA, 45 bp, Homo sapiens
tgtgtggtgaagccggcatcaggaggaagctacatacctacattt

SEQ ID NO: 649 - DNA, 45 bp, Homo sapiens
tgtgtggtccgccgcgcatcaggaggaagctacatacctacattt

SEQ ID NO: 650 - DNA, 45 bp, Homo sapiens
tgtgtggtctctcttgcatcaggaggaagctacatacctacattt

SEQ ID NO: 651 - DNA, 45 bp, Homo sapiens
tgtgtggtgagtatagcatcaggaggaagctacatacctacattt

SEQ ID NO: 652 - DNA, 45 bp, Homo sapiens
tgtgtggtgaatagcgcgggaggaggaagctacatacctacattt

SEQ ID NO: 653 - DNA, 45 bp, Homo sapiens
tgtgtggtgaacgtggcaggaggaggaagctacatacctacattt

SEQ ID NO: 654 - DNA, 45 bp, Homo sapiens
tgtgtggtgtctttggcatcaggaggaagctacatacctacattt

SEQ ID NO: 655 - DNA, 45 bp, Homo sapiens
tgtgtggtgtcttctgcatcaggaggaagctacatacctacattt

SEQ ID NO: 656 - DNA, 45 bp, Homo sapiens
tgtgtggtgagcactgcatcaggaggaagctacatacctacattt

SEQ ID NO: 657 - DNA, 45 bp, Homo sapiens
tgtgtggtgtggggggcatcaggaggaagctacatacctacattt

SEQ ID NO: 658 - DNA, 45 bp, Homo sapiens
tgtgtggtgaccacagccggaggaggaagctacatacctacattt

SEQ ID NO: 659 - DNA, 45 bp, Homo sapiens
tgtgtggtgaacctcgcggcaggaggaagctacatacctacattt

SEQ ID NO: 660 - DNA, 45 bp, Homo sapiens
tgtgtggtccgactcgcatcaggaggaagctacatacctacattt

SEQ ID NO: 661 - DNA, 45 bp, Homo sapiens
tgtgtggtgtccggcgcatcaggaggaagctacatacctacattt

SEQ ID NO: 662 - DNA, 45 bp, Homo sapiens
tgtgtggtgagttccgcatcaggaggaagctacatacctacattt

SEQ ID NO: 663 - DNA, 45 bp, Homo sapiens
tgtgtggtgaaccttgcggcaggaggaagctacatacctacattt

SEQ ID NO: 664 - DNA, 45 bp, Homo sapiens
tgtgtggtgcgtctagcatcaggaggaagctacatacctacattt

SEQ ID NO: 665 - DNA, 45 bp, Homo sapiens
tgtgtggtgatccatgcatcaggaggaagctacatacctacattt

SEQ ID NO: 666 - DNA, 45 bp, Homo sapiens
tgtgtggtccatcttgcatcaggaggaagctacatacctacattt

SEQ ID NO: 667 - DNA, 45 bp, Homo sapiens
tgtgtggtgactccggcatcaggaggaagctacatacctacattt

SEQ ID NO: 668 - DNA, 45 bp, Homo sapiens
tgtgtggtgttttcggcatcaggaggaagctacatacctacattt

SEQ ID NO: 669 - DNA, 45 bp, Homo sapiens
tgtgtggtgaacgtagcagggggaggaagctacatacctacattt

SEQ ID NO: 670 - DNA, 45 bp, Homo sapiens
tgtgtggtgactttggcatcaggaggaagctacatacctacattt

SEQ ID NO: 671 - DNA, 45 bp, Homo sapiens
tgtgtggtgatccttgcatcaggaggaagctacatacctacattt

SEQ ID NO: 672 - DNA, 45 bp, Homo sapiens
tgtgtggtgatccccgcgacaggaggaagctacatacctacattt

SEQ ID NO: 673 - DNA, 45 bp, Homo sapiens
tgtgtggtgaccgttgcatcaggaggaagctacatacctacattt

SEQ ID NO: 674 - DNA, 45 bp, Homo sapiens
tgtgtggtgaacatggctggaggaggaagctacatacctacattt

SEQ ID NO: 675 - DNA, 45 bp, Homo sapiens
tgtgtggtgaagacagcatcaggaggaagctacatacctacattt

SEQ ID NO: 676 - DNA, 45 bp, Homo sapiens
tgtgtggtacacgaggcatcaggaggaagctacatacctacattt

SEQ ID NO: 677 - DNA, 45 bp, Homo sapiens
tgtgtggtccctcatgcatcaggaggaagctacatacctacattt

SEQ ID NO: 678 - DNA, 45 bp, Homo sapiens
tgtgtggtgatcattgcatcaggaggaagctacatacctacattt

SEQ ID NO: 679 - DNA, 45 bp, Homo sapiens
tgtgtggtttggccggcatcaggaggaagctacatacctacattt

SEQ ID NO: 680 - DNA, 45 bp, Homo sapiens
tgtgtggtgagtcctgcatcaggaggaagctacatacctacattt

SEQ ID NO: 681 - DNA, 45 bp, Homo sapiens
tgtgtggtgaaccctgcttcaggaggaagctacatacctacattt

SEQ ID NO: 682 - DNA, 45 bp, Homo sapiens
tgtgtggtgaacggggcttcaggaggaagctacatacctacattt

SEQ ID NO: 683 - DNA, 45 bp, Homo sapiens
tgtgtggtgatcggtgcatcaggaggaagctacatacctacattt

SEQ ID NO: 684 - DNA, 45 bp, Homo sapiens
tgtgtggtgagccccgcatcaggaggaagctacatacctacattt

SEQ ID NO: 685 - DNA, 45 bp, Homo sapiens
tgtgtggtgaacgcagcatcaggaggaagctacatacctacattt

SEQ ID NO: 686 - DNA, 45 bp, Homo sapiens
tgtgtggtggccttcgcatcaggaggaagctacatacctacattt

SEQ ID NO: 687 - DNA, 45 bp, Homo sapiens
tgtgtggtgaacaccgcgggaggaggaagctacatacctacattt

SEQ ID NO: 688 - DNA, 45 bp, Homo sapiens
tgtgtggtccggatagcatcaggaggaagctacatacctacattt

SEQ ID NO: 689 - DNA, 45 bp, Homo sapiens
tgtgtggtgatggccgcatcaggaggaagctacatacctacattt

SEQ ID NO: 690 - DNA, 45 bp, Homo sapiens
tgtgtggtgaacaaggccgcgggaggaagctacatacctacattt

SEQ ID NO: 691 - DNA, 45 bp, Homo sapiens
tgtgtggtgacccatgcatcaggaggaagctacatacctacattt

SEQ ID NO: 692 - DNA, 45 bp, Homo sapiens
tgtgtggtgaccttagcatcaggaggaagctacatacctacattt

SEQ ID NO: 693 - DNA, 45 bp, Homo sapiens
tgtgtggtgaacgtggcggcaggaggaagctacatacctacattt

SEQ ID NO: 694 - DNA, 45 bp, Homo sapiens
tgtgtggtgaggttcgcatcaggaggaagctacatacctacattt

SEQ ID NO: 695 - DNA, 45 bp, Homo sapiens
tgtgtggtgtcctttgcatcaggaggaagctacatacctacattt

SEQ ID NO: 696 - DNA, 45 bp, Homo sapiens
tgtgtggtgaggtatgcatcaggaggaagctacatacctacattt

SEQ ID NO: 697 - DNA, 45 bp, Homo sapiens
tgtgtggtgaggcatgcaacaggaggaagctacatacctacattt

SEQ ID NO: 698 - DNA, 45 bp, Homo sapiens
tgtgtggtgagggtagcatcaggaggaagctacatacctacattt

SEQ ID NO: 699 - DNA, 45 bp, Homo sapiens
tgtgtggtgaactcggcagcaggaggaagctacatacctacattt

SEQ ID NO: 700 - DNA, 45 bp, Homo sapiens
tgtgtggtgaacgtagcagcaggaggaagctacatacctacattt

SEQ ID NO: 701 - DNA, 45 bp, Homo sapiens
tgtgtggtgaacatggccacaggaggaagctacatacctacattt

SEQ ID NO: 702 - DNA, 45 bp, Homo sapiens
tgtgtggtacgtcgggcatcaggaggaagctacatacctacattt

SEQ ID NO: 703 - DNA, 45 bp, Homo sapiens
tgtgtggtcgctacggcatcaggaggaagctacatacctacattt

SEQ ID NO: 704 - DNA, 45 bp, Homo sapiens
tgtgtggtttcccatgcatcaggaggaagctacatacctacattt

SEQ ID NO: 705 - DNA, 45 bp, Homo sapiens
tgtgtggtgaacggtgcatcaggaggaagctacatacctacattt

SEQ ID NO: 706 - DNA, 45 bp, Homo sapiens
tgtgtggtgcggaccgcatcaggaggaagctacatacctacattt

SEQ ID NO: 707 - DNA, 45 bp, Homo sapiens
tgtgtggtgtcaaaagcatcaggaggaagctacatacctacattt

SEQ ID NO: 708 - DNA, 45 bp, Homo sapiens
tgtgtggtggccttagcatcaggaggaagctacatacctacattt

SEQ ID NO: 709 - DNA, 45 bp, Homo sapiens
tgtgtggtgaacatcgccgcaggaggaagctacatacctacattt

SEQ ID NO: 710 - DNA, 45 bp, Homo sapiens
tgtgtggttcgggaggcatcaggaggaagctacatacctacattt

SEQ ID NO: 711 - DNA, 45 bp, Homo sapiens
tgtgtggttgctcatgcatcaggaggaagctacatacctacattt

SEQ ID NO: 712 - DNA, 45 bp, Homo sapiens
tgtgtggtgaaagtagctggtggaggaagctacatacctacattt

SEQ ID NO: 713 - DNA, 45 bp, Homo sapiens
tgtgtggtgcgtactgcatcaggaggaagctacatacctacattt

SEQ ID NO: 714 - DNA, 45 bp, Homo sapiens
tgtgtggtgaacctcgcgggaggaggaagctacatacctacattt

SEQ ID NO: 715 - DNA, 45 bp, Homo sapiens
tgtgtggtgaacatagcgggaggaggaagctacatacctacattt

SEQ ID NO: 716 - DNA, 45 bp, Homo sapiens
tgtgtggtgagtctggcatcaggaggaagctacatacctacattt

SEQ ID NO: 717 - DNA, 45 bp, Homo sapiens
tgtgtggtgagagcagcatcaggaggaagctacatacctacattt

SEQ ID NO: 718 - DNA, 45 bp, Homo sapiens
tgtgtggtgaacaaagccccaggaggaagctacatacctacattt

SEQ ID NO: 719 - DNA, 45 bp, Homo sapiens
tgtgtggtccctttcgcatcaggaggaagctacatacctacattt

SEQ ID NO: 720 - DNA, 45 bp, Homo sapiens
tgtgtggtgtccctcgcatcaggaggaagctacatacctacattt

SEQ ID NO: 721 - DNA, 45 bp, Homo sapiens
tgtgtggtgtcgtctgcatcaggaggaagctacatacctacattt

SEQ ID NO: 722 - DNA, 45 bp, Homo sapiens
tgtgtggtgccggtagcatcaggaggaagctacatacctacattt

SEQ ID NO: 723 - DNA, 45 bp, Homo sapiens
tgtgtggtgcgacgcgcatcaggaggaagctacatacctacattt

SEQ ID NO: 724 - DNA, 45 bp, Homo sapiens
tgtgtggtgagtcaggcatcaggaggaagctacatacctacattt

SEQ ID NO: 725 - DNA, 45 bp, Homo sapiens
tgtgtggtgagggtcgccggaggaggaagctacatacctacattt

SEQ ID NO: 726 - DNA, 45 bp, Homo sapiens
tgtgtggtgagggcagcatcaggaggaagctacatacctacattt

SEQ ID NO: 727 - DNA, 45 bp, Homo sapiens
tgtgtggtgaggactgcatcaggaggaagctacatacctacattt

SEQ ID NO: 728 - DNA, 45 bp, Homo sapiens
tgtgtggtgagaaccgcccaaggaggaagctacatacctacattt

SEQ ID NO: 729 - DNA, 45 bp, Homo sapiens
tgtgtggtgaatattgcatcaggaggaagctacatacctacattt

SEQ ID NO: 730 - DNA, 45 bp, Homo sapiens
tgtgtggtgaacacggcgggaggaggaagctacatacctacattt

SEQ ID NO: 731 - DNA, 45 bp, Homo sapiens
tgtgtggtggcctccgcatcaggaggaagctacatacctacattt

SEQ ID NO: 732 - DNA, 45 bp, Homo sapiens
tgtgtggtgaggtcggcatcaggaggaagctacatacctacattt

SEQ ID NO: 733 - DNA, 45 bp, Homo sapiens
tgtgtggtgaggcgcgcatcaggaggaagctacatacctacattt

SEQ ID NO: 734 - DNA, 45 bp, Homo sapiens
tgtgtggtccgacaggcatcaggaggaagctacatacctacattt

SEQ ID NO: 735 - DNA, 45 bp, Homo sapiens
tgtgtggtgggcctcgcatcaggaggaagctacatacctacattt

SEQ ID NO: 736 - DNA, 45 bp, Homo sapiens
tgtgtggtgaccagcgctacaggaggaagctacatacctacattt

SEQ ID NO: 737 - DNA, 45 bp, Homo sapiens
tgtgtggtgttcctcgcatcaggaggaagctacatacctacattt

SEQ ID NO: 738 - DNA, 45 bp, Homo sapiens
tgtgtggtgagtggagcatcaggaggaagctacatacctacattt

SEQ ID NO: 739 - DNA, 45 bp, Homo sapiens
tgtgtggtgagggtcgcagcaggaggaagctacatacctacattt

SEQ ID NO: 740 - DNA, 45 bp, Homo sapiens
tgtgtggtgacctcagcatcaggaggaagctacatacctacattt

SEQ ID NO: 741 - DNA, 45 bp, Homo sapiens
tgtgtggtgaacctggcggcaggaggaagctacatacctacattt

SEQ ID NO: 742 - DNA, 45 bp, Homo sapiens
tgtgtggtgaacgtggcatcaggaggaagctacatacctacattt

SEQ ID NO: 743 - DNA, 45 bp, Homo sapiens
tgtgtggtgaagacggcatcaggaggaagctacatacctacattt

SEQ ID NO: 744 - DNA, 45 bp, Homo sapiens
tgtgtggtgtccttcgcctcaggaggaagctacatacctacattt

SEQ ID NO: 745 - DNA, 45 bp, Homo sapiens
tgtgtggtgagcggtgcatcaggaggaagctacatacctacattt

SEQ ID NO: 746 - DNA, 45 bp, Homo sapiens
tgtgtggtgcgcctagcatcaggaggaagctacatacctacattt

SEQ ID NO: 747 - DNA, 45 bp, Homo sapiens
tgtgtggtgagtctagcatcaggaggaagctacatacctacattt

SEQ ID NO: 748 - DNA, 45 bp, Homo sapiens
tgtgtggtgaacggggccccaggaggaagctacatacctacattt

SEQ ID NO: 749 - DNA, 45 bp, Homo sapiens
tgtgtggtgaacggggcccaaggaggaagctacatacctacattt

SEQ ID NO: 750 - DNA, 45 bp, Homo sapiens
tgtgtggtgaaaatggcatcaggaggaagctacatacctacattt

SEQ ID NO: 751 - DNA, 45 bp, Homo sapiens
tgtgtggtgaaccccgcgtcaggaggaagctacatacctacattt

SEQ ID NO: 752 - DNA, 45 bp, Homo sapiens
tgtgtggtgcgccttgcatcaggaggaagctacatacctacattt

SEQ ID NO: 753 - DNA, 45 bp, Homo sapiens
tgtgtggtacgccatgcatcaggaggaagctacatacctacattt

SEQ ID NO: 754 - DNA, 45 bp, Homo sapiens
tgtgtggtgttcctagcatcaggaggaagctacatacctacattt

SEQ ID NO: 755 - DNA, 45 bp, Homo sapiens
tgtgtggtgaacctcgcccgaggaggaagctacatacctacattt

SEQ ID NO: 756 - DNA, 45 bp, Homo sapiens
tgtgtggtcgctcccgcatcaggaggaagctacatacctacattt

SEQ ID NO: 757 - DNA, 45 bp, Homo sapiens
tgtgtggtgcttggggccgcaggaggaagctacatacctacattt

SEQ ID NO: 758 - DNA, 45 bp, Homo sapiens
tgtgtggtgctcggcgcatcaggaggaagctacatacctacattt

SEQ ID NO: 759 - DNA, 45 bp, Homo sapiens
tgtgtggtgatgggtgcatcaggaggaagctacatacctacattt

SEQ ID NO: 760 - DNA, 45 bp, Homo sapiens
tgtgtggtgagattagcatcaggaggaagctacatacctacattt

SEQ ID NO: 761 - DNA, 45 bp, Homo sapiens
tgtgtggttccccatgcatcaggaggaagctacatacctacattt

SEQ ID NO: 762 - DNA, 45 bp, Homo sapiens
tgtgtggtgaccgatgcatcaggaggaagctacatacctacattt

SEQ ID NO: 763 - DNA, 45 bp, Homo sapiens
tgtgtggtgaccgacgcatcaggaggaagctacatacctacattt

SEQ ID NO: 764 - DNA, 45 bp, Homo sapiens
tgtgtggtgaacaaggcgacaggaggaagctacatacctacattt

SEQ ID NO: 765 - DNA, 45 bp, Homo sapiens
tgtgtggtgaatcgggcatcaggaggaagctacatacctacattt

SEQ ID NO: 766 - DNA, 45 bp, Homo sapiens
tgtgtggtgaagggggcctcaggaggaagctacatacctacattt

SEQ ID NO: 767 - DNA, 45 bp, Homo sapiens
tgtgtggtggtaggggcatcaggaggaagctacatacctacattt

SEQ ID NO: 768 - DNA, 45 bp, Homo sapiens
tgtgtggtggatcatgcatcaggaggaagctacatacctacattt

SEQ ID NO: 769 - DNA, 45 bp, Homo sapiens
tgtgtggtgttagttgcatcaggaggaagctacatacctacattt

SEQ ID NO: 770 - DNA, 45 bp, Homo sapiens
tgtgtggtgacccaagcatcaggaggaagctacatacctacattt

SEQ ID NO: 771 - DNA, 45 bp, Homo sapiens
tgtgtggtgaggatagcatcaggaggaagctacatacctacattt

SEQ ID NO: 772 - DNA, 45 bp, Homo sapiens
tgtgtggtgactgccgcatcaggaggaagctacatacctacattt

SEQ ID NO: 773 - DNA, 45 bp, Homo sapiens
tgtgtggtgtcccccgcatcaggaggaagctacatacctacattt

SEQ ID NO: 774 - DNA, 45 bp, Homo sapiens
tgtgtggtgattcctgcatcaggaggaagctacatacctacattt

SEQ ID NO: 775 - DNA, 45 bp, Homo sapiens
tgtgtggtgaaggcagcatcaggaggaagctacatacctacattt

SEQ ID NO: 776 - DNA, 45 bp, Homo sapiens
tgtgtggtgaggcgggcatcaggaggaagctacatacctacattt

SEQ ID NO: 777 - DNA, 45 bp, Homo sapiens
tgtgtggtgagcctggcatcaggaggaagctacatacctacattt

SEQ ID NO: 778 - DNA, 45 bp, Homo sapiens
tgtgtggtgaatttggcatcaggaggaagctacatacctacattt

SEQ ID NO: 779 - DNA, 45 bp, Homo sapiens
tgtgtggtgaacagagcaccaggaggaagctacatacctacattt

SEQ ID NO: 780 - DNA, 45 bp, Homo sapiens
tgtgtggtgattccggcatcaggaggaagctacatacctacattt

SEQ ID NO: 781 - DNA, 45 bp, Homo sapiens
tgtgtggtgattaccgcatcaggaggaagctacatacctacattt

SEQ ID NO: 782 - DNA, 45 bp, Homo sapiens
tgtgtggtgattctagcatcaggaggaagctacatacctacattt

SEQ ID NO: 783 - DNA, 45 bp, Homo sapiens
tgtgtggtgatctctgcatcaggaggaagctacatacctacattt

SEQ ID NO: 784 - DNA, 45 bp, Homo sapiens
tgtgtggtgaatcctgcatcaggaggaagctacatacctacattt

SEQ ID NO: 785 - DNA, 45 bp, Homo sapiens
tgtgtggtgaacttggcttcaggaggaagctacatacctacattt

SEQ ID NO: 786 - DNA, 45 bp, Homo sapiens
tgtgtggtgaacatcgctgcaggaggaagctacatacctacattt

SEQ ID NO: 787 - DNA, 45 bp, Homo sapiens
tgtgtggtgaacccagcctcaggaggaagctacatacctacattt

SEQ ID NO: 788 - DNA, 45 bp, Homo sapiens
tgtgtggtgaaccacgcatcaggaggaagctacatacctacattt

SEQ ID NO: 789 - DNA, 45 bp, Homo sapiens
tgtgtggtcctgcatgcatcaggaggaagctacatacctacattt

SEQ ID NO: 790 - DNA, 45 bp, Homo sapiens
tgtgtggtgattctcgcatcaggaggaagctacatacctacattt

SEQ ID NO: 791 - DNA, 45 bp, Homo sapiens
tgtgtggtgattggggcatcaggaggaagctacatacctacattt

SEQ ID NO: 792 - DNA, 45 bp, Homo sapiens
tgtgtggtgaacggggcgcgaggaggaagctacatacctacattt

SEQ ID NO: 793 - DNA, 45 bp, Homo sapiens
tgtgtggtgataggtgcatcaggaggaagctacatacctacattt

SEQ ID NO: 794 - DNA, 45 bp, Homo sapiens
tgtgtggtgaccggcgcatcaggaggaagctacatacctacattt

SEQ ID NO: 795 - DNA, 45 bp, Homo sapiens
tgtgtggtgaaccgggcggcaggaggaagctacatacctacattt

SEQ ID NO: 796 - DNA, 45 bp, Homo sapiens
tgtgtggtgcgtctcgcatcaggaggaagctacatacctacattt

SEQ ID NO: 797 - DNA, 45 bp, Homo sapiens
tgtgtggtggccgatgcatcaggaggaagctacatacctacattt

SEQ ID NO: 798 - DNA, 45 bp, Homo sapiens
tgtgtggtgactcatgcatcaggaggaagctacatacctacattt

SEQ ID NO: 799 - DNA, 45 bp, Homo sapiens
tgtgtggtgaacatcgcaccaggaggaagctacatacctacattt

SEQ ID NO: 800 - DNA, 45 bp, Homo sapiens
tgtgtggtgaggagcgcatcaggaggaagctacatacctacattt

SEQ ID NO: 801 - DNA, 45 bp, Homo sapiens
tgtgtggtgatcgctgcatcaggaggaagctacatacctacattt

SEQ ID NO: 802 - DNA, 45 bp, Homo sapiens
tgtgtggtgaacagcgcggcaggaggaagctacatacctacattt

SEQ ID NO: 803 - DNA, 45 bp, Homo sapiens
tgtgtggtgccgcatgcatcaggaggaagctacatacctacattt

SEQ ID NO: 804 - DNA, 45 bp, Homo sapiens
tgtgtggtgaacccggctccaggaggaagctacatacctacattt

SEQ ID NO: 805 - DNA, 45 bp, Homo sapiens
tgtgtggtgagaggtgcatcaggaggaagctacatacctacattt

SEQ ID NO: 806 - DNA, 45 bp, Homo sapiens
tgtgtggtgaaggctgcatcaggaggaagctacatacctacattt

SEQ ID NO: 807 - DNA, 45 bp, Homo sapiens
tgtgtggtgatcctcgcatcaggaggaagctacatacctacattt

SEQ ID NO: 808 - DNA, 45 bp, Homo sapiens
tgtgtggtgaacggggcggggggaggaagctacatacctacattt

SEQ ID NO: 809 - DNA, 45 bp, Homo sapiens
tgtgtggtgaacaaggcgaaaggaggaagctacatacctacattt

SEQ ID NO: 810 - DNA, 45 bp, Homo sapiens
tgtgtggtgaaactggccgtcggaggaagctacatacctacattt

SEQ ID NO: 811 - DNA, 45 bp, Homo sapiens
tgtgtggtgaaaggcgcatcaggaggaagctacatacctacattt

SEQ ID NO: 812 - DNA, 45 bp, Homo sapiens
tgtgtggtgaagagggcggggggaggaagctacatacctacattt

SEQ ID NO: 813 - DNA, 45 bp, Homo sapiens
tgtgtggtgaacgctgccaggggaggaagctacatacctacattt

SEQ ID NO: 814 - DNA, 45 bp, Homo sapiens
tgtgtggttcattatgcatcaggaggaagctacatacctacattt

SEQ ID NO: 815 - DNA, 45 bp, Homo sapiens
tgtgtggtggctcatgcatcaggaggaagctacatacctacattt

SEQ ID NO: 816 - DNA, 45 bp, Homo sapiens
tgtgtggtccagagtgcatcaggaggaagctacatacctacattt

SEQ ID NO: 817 - DNA, 45 bp, Homo sapiens
tgtgtggtgttccttgcatcaggaggaagctacatacctacattt

SEQ ID NO: 818 - DNA, 45 bp, Homo sapiens
tgtgtggtgtccttggcatcaggaggaagctacatacctacattt

SEQ ID NO: 819 - DNA, 45 bp, Homo sapiens
tgtgtggtggtccgagcatcaggaggaagctacatacctacattt

SEQ ID NO: 820 - DNA, 45 bp, Homo sapiens
tgtgtggtgattgtagcatcaggaggaagctacatacctacattt

SEQ ID NO: 821 - DNA, 45 bp, Homo sapiens
tgtgtggtgaactctgcgtcaggaggaagctacatacctacattt

SEQ ID NO: 822 - DNA, 45 bp, Homo sapiens
tgtgtggtgaacggggcagcaggaggaagctacatacctacattt

SEQ ID NO: 823 - DNA, 45 bp, Homo sapiens
tgtgtggtggggaccgcatcaggaggaagctacatacctacattt

SEQ ID NO: 824 - DNA, 45 bp, Homo sapiens
tgtgtggtgaacggagccccaggaggaagctacatacctacattt

SEQ ID NO: 825 - DNA, 45 bp, Homo sapiens
tgtgtggtgattatcgcatcaggaggaagctacatacctacattt

SEQ ID NO: 826 - DNA, 45 bp, Homo sapiens
tgtgtggtgtctcgggccatgggaggaagctacatacctacattt

SEQ ID NO: 827 - DNA, 45 bp, Homo sapiens
tgtgtggtgaagaacgcatcaggaggaagctacatacctacattt

SEQ ID NO: 828 - DNA, 45 bp, Homo sapiens
tgtgtggtgcttcatgcatcaggaggaagctacatacctacattt

SEQ ID NO: 829 - DNA, 45 bp, Homo sapiens
tgtgtggtgaccgccgcatcaggaggaagctacatacctacattt

SEQ ID NO: 830 - DNA, 45 bp, Homo sapiens
tgtgtggtgaaacatgcatcaggaggaagctacatacctacattt

SEQ ID NO: 831 - DNA, 45 bp, Homo sapiens
tgtgtggtttcccttgcagcaggaggaagctacatacctacattt

SEQ ID NO: 832 - DNA, 45 bp, Homo sapiens
tgtgtggtgatgaccgcatcaggaggaagctacatacctacattt

SEQ ID NO: 833 - DNA, 45 bp, Homo sapiens
tgtgtggtgacgcatgcatcaggaggaagctacatacctacattt

SEQ ID NO: 834 - DNA, 45 bp, Homo sapiens
tgtgtggtgagctttgcatcaggaggaagctacatacctacattt

SEQ ID NO: 835 - DNA, 45 bp, Homo sapiens
tgtgtggtgaaaagggcatcaggaggaagctacatacctacattt

SEQ ID NO: 836 - DNA, 45 bp, Homo sapiens
tgtgtggtgaaacgggcatcaggaggaagctacatacctacattt

SEQ ID NO: 837 - DNA, 45 bp, Homo sapiens
tgtgtggtgaccggtgcatcaggaggaagctacatacctacattt

SEQ ID NO: 838 - DNA, 45 bp, Homo sapiens
tgtgtggtgaaaggagcatcaggaggaagctacatacctacattt

SEQ ID NO: 839 - DNA, 45 bp, Homo sapiens
tgtgtggtgatgctggcatcaggaggaagctacatacctacattt

SEQ ID NO: 840 - DNA, 45 bp, Homo sapiens
tgtgtggtgaacgaggcaacaggaggaagctacatacctacattt

SEQ ID NO: 841 - DNA, 45 bp, Homo sapiens
tgtgtggtgtcccgcgcctcaggaggaagctacatacctacattt

SEQ ID NO: 842 - DNA, 45 bp, Homo sapiens
tgtgtggtgacgctggcatcaggaggaagctacatacctacattt

SEQ ID NO: 843 - DNA, 45 bp, Homo sapiens
tgtgtggtgaacatggccccaggaggaagctacatacctacattt

SEQ ID NO: 844 - DNA, 45 bp, Homo sapiens
tgtgtggtgttacccgcatcaggaggaagctacatacctacattt

SEQ ID NO: 845 - DNA, 45 bp, Homo sapiens
tgtgtggtgaataccgcatcaggaggaagctacatacctacattt

SEQ ID NO: 846 - DNA, 45 bp, Homo sapiens
tgtgtggtgaactatgcatcaggaggaagctacatacctacattt

SEQ ID NO: 847 - DNA, 45 bp, Homo sapiens
tgtgtggttccctttgcatcaggaggaagctacatacctacattt

SEQ ID NO: 848 - DNA, 45 bp, Homo sapiens
tgtgtggttttcggtgcatcaggaggaagctacatacctacattt

SEQ ID NO: 849 - DNA, 45 bp, Homo sapiens
tgtgtggtgagacaggcatcaggaggaagctacatacctacattt

SEQ ID NO: 850 - DNA, 45 bp, Homo sapiens
tgtgtggttcagggggcatcaggaggaagctacatacctacattt

SEQ ID NO: 851 - DNA, 45 bp, Homo sapiens
tgtgtggtgaggcctgcatcaggaggaagctacatacctacattt

SEQ ID NO: 852 - DNA, 45 bp, Homo sapiens
tgtgtggtgaatggggcctcaggaggaagctacatacctacattt

SEQ ID NO: 853 - DNA, 45 bp, Homo sapiens
tgtgtggtgaactccgcctcaggaggaagctacatacctacattt

SEQ ID NO: 854 - DNA, 45 bp, Homo sapiens
tgtgtggtccgaatggcatcaggaggaagctacatacctacattt

SEQ ID NO: 855 - DNA, 45 bp, Homo sapiens
tgtgtggtgaggtctgcatcaggaggaagctacatacctacattt

SEQ ID NO: 856 - DNA, 45 bp, Homo sapiens
tgtgtggtgagggcggcatcaggaggaagctacatacctacattt

SEQ ID NO: 857 - DNA, 45 bp, Homo sapiens
tgtgtggtgaacatggcccccggaggaagctacatacctacattt

SEQ ID NO: 858 - DNA, 45 bp, Homo sapiens
tgtgtggtgatctcggcatcaggaggaagctacatacctacattt

SEQ ID NO: 859 - DNA, 45 bp, Homo sapiens
tgtgtggtgattgttgcatcaggaggaagctacatacctacattt

SEQ ID NO: 860 - DNA, 45 bp, Homo sapiens
tgtgtggtgacgtccgcatcaggaggaagctacatacctacattt

SEQ ID NO: 861 - DNA, 45 bp, Homo sapiens
tgtgtggtgaactgggcgggaggaggaagctacatacctacattt

SEQ ID NO: 862 - DNA, 45 bp, Homo sapiens
tgtgtggtgacctccgcatcaggaggaagctacatacctacattt

SEQ ID NO: 863 - DNA, 45 bp, Homo sapiens
tgtgtggttacatatgcatcaggaggaagctacatacctacattt

SEQ ID NO: 864 - DNA, 45 bp, Homo sapiens
tgtgtggtctacggagcatcaggaggaagctacatacctacattt

SEQ ID NO: 865 - DNA, 45 bp, Homo sapiens
tgtgtggtgaccttggcatcaggaggaagctacatacctacattt

SEQ ID NO: 866 - DNA, 45 bp, Homo sapiens
tgtgtggtgagtcccgcatcaggaggaagctacatacctacattt

SEQ ID NO: 867 - DNA, 45 bp, Homo sapiens
tgtgtggtcggcgatgcatcaggaggaagctacatacctacattt

SEQ ID NO: 868 - DNA, 45 bp, Homo sapiens
tgtgtggtgaacacagctcgaggaggaagctacatacctacattt

SEQ ID NO: 869 - DNA, 45 bp, Homo sapiens
tgtgtggtctacttggcatcaggaggaagctacatacctacattt

SEQ ID NO: 870 - DNA, 45 bp, Homo sapiens
tgtgtggtggttcatgcatcaggaggaagctacatacctacattt

SEQ ID NO: 871 - DNA, 45 bp, Homo sapiens
tgtgtggtgagtacagcatcaggaggaagctacatacctacattt

SEQ ID NO: 872 - DNA, 45 bp, Homo sapiens
tgtgtggtgaaccaggccacaggaggaagctacatacctacattt

SEQ ID NO: 873 - DNA, 45 bp, Homo sapiens
tgtgtggtgatcaccgcatcaggaggaagctacatacctacattt

SEQ ID NO: 874 - DNA, 45 bp, Homo sapiens
tgtgtggtgaacagagcgtcaggaggaagctacatacctacattt

SEQ ID NO: 875 - DNA, 45 bp, Homo sapiens
tgtgtggtgcgtcaagcatcaggaggaagctacatacctacattt

SEQ ID NO: 876 - DNA, 45 bp, Homo sapiens
tgtgtggtgcgcggagcatcaggaggaagctacatacctacattt

SEQ ID NO: 877 - DNA, 45 bp, Homo sapiens
tgtgtggtggcctgggcatcaggaggaagctacatacctacattt

SEQ ID NO: 878 - DNA, 45 bp, Homo sapiens
tgtgtggtgaggggtgcatcaggaggaagctacatacctacattt

SEQ ID NO: 879 - DNA, 45 bp, Homo sapiens
tgtgtggtgaacggggcaccaggaggaagctacatacctacattt

SEQ ID NO: 880 - DNA, 45 bp, Homo sapiens
tgtgtggtgaatttagcatcaggaggaagctacatacctacattt

SEQ ID NO: 881 - DNA, 45 bp, Homo sapiens
tgtgtggtgtggaccgcatcaggaggaagctacatacctacattt

SEQ ID NO: 882 - DNA, 45 bp, Homo sapiens
tgtgtggtgctacatgcatcaggaggaagctacatacctacattt

SEQ ID NO: 883 - DNA, 45 bp, Homo sapiens
tgtgtggtgagactcgcatcaggaggaagctacatacctacattt

SEQ ID NO: 884 - DNA, 45 bp, Homo sapiens
tgtgtggtgattgctgcatcaggaggaagctacatacctacattt

SEQ ID NO: 885 - DNA, 45 bp, Homo sapiens
tgtgtggtgatctacgcatcaggaggaagctacatacctacattt

SEQ ID NO: 886 - DNA, 45 bp, Homo sapiens
tgtgtggtgactatcgcatcaggaggaagctacatacctacattt

SEQ ID NO: 887 - DNA, 45 bp, Homo sapiens
tgtgtggttcctcccgcatcaggaggaagctacatacctacattt

SEQ ID NO: 888 - DNA, 45 bp, Homo sapiens
tgtgtggttagactcgcatcaggaggaagctacatacctacattt

SEQ ID NO: 889 - DNA, 45 bp, Homo sapiens
tgtgtggtggaccatgcatcaggaggaagctacatacctacattt

SEQ ID NO: 890 - DNA, 45 bp, Homo sapiens
tgtgtggtgattcacgcatcaggaggaagctacatacctacattt

SEQ ID NO: 891 - DNA, 45 bp, Homo sapiens
tgtgtggtggacgacgcatcaggaggaagctacatacctacattt

SEQ ID NO: 892 - DNA, 45 bp, Homo sapiens
tgtgtggtgaagggggccccaggaggaagctacatacctacattt

SEQ ID NO: 893 - DNA, 45 bp, Homo sapiens
tgtgtggtctaccccgcatcaggaggaagctacatacctacattt

SEQ ID NO: 894 - DNA, 45 bp, Homo sapiens
tgtgtggtgccgccagctccaggaggaagctacatacctacattt

SEQ ID NO: 895 - DNA, 45 bp, Homo sapiens
tgtgtggtgtcccaggcatcaggaggaagctacatacctacattt

SEQ ID NO: 896 - DNA, 45 bp, Homo sapiens
tgtgtggtgattttcgcatcaggaggaagctacatacctacattt

SEQ ID NO: 897 - DNA, 45 bp, Homo sapiens
tgtgtggtgatcctggcatcaggaggaagctacatacctacattt

SEQ ID NO: 898 - DNA, 45 bp, Homo sapiens
tgtgtggtgatcccggcgtcaggaggaagctacatacctacattt

SEQ ID NO: 899 - DNA, 45 bp, Homo sapiens
tgtgtggtgactcccgcatcaggaggaagctacatacctacattt

SEQ ID NO: 900 - DNA, 45 bp, Homo sapiens
tgtgtggtgaaccgggccccaggaggaagctacatacctacattt

SEQ ID NO: 901 - DNA, 45 bp, Homo sapiens
tgtgtggtgaactcggccgaagggggaagctacatacctacattt

SEQ ID NO: 902 - DNA, 45 bp, Homo sapiens
tgtgtggtcctccatgcatcaggaggaagctacatacctacattt

SEQ ID NO: 903 - DNA, 45 bp, Homo sapiens
tgtgtggtgttaggggcatcaggaggaagctacatacctacattt

SEQ ID NO: 904 - DNA, 45 bp, Homo sapiens
tgtgtggtgtactttgcatcaggaggaagctacatacctacattt

SEQ ID NO: 905 - DNA, 45 bp, Homo sapiens
tgtgtggtgaacgaggcgtcaggaggaagctacatacctacattt

SEQ ID NO: 906 - DNA, 45 bp, Homo sapiens
tgtgtggtgaacaacgcatcaggaggaagctacatacctacattt

SEQ ID NO: 907 - DNA, 45 bp, Homo sapiens
tgtgtggtgagtttcgcatcaggaggaagctacatacctacattt

SEQ ID NO: 908 - DNA, 45 bp, Homo sapiens
tgtgtggtgaaccgagcggcaggaggaagctacatacctacattt

SEQ ID NO: 909 - DNA, 45 bp, Homo sapiens
tgtgtggtgaacggcgctccaggaggaagctacatacctacattt

SEQ ID NO: 910 - DNA, 45 bp, Homo sapiens
tgtgtggtgaacatggcgccaggaggaagctacatacctacattt

SEQ ID NO: 911 - DNA, 45 bp, Homo sapiens
tgtgtggtccgatccgcatcaggaggaagctacatacctacattt

SEQ ID NO: 912 - DNA, 45 bp, Homo sapiens
tgtgtggtgattttggcatcaggaggaagctacatacctacattt

SEQ ID NO: 913 - DNA, 45 bp, Homo sapiens
tgtgtggtgagcgcagcatcaggaggaagctacatacctacattt

SEQ ID NO: 914 - DNA, 45 bp, Homo sapiens
tgtgtggtgaactcagcaaaaggaggaagctacatacctacattt

SEQ ID NO: 915 - DNA, 45 bp, Homo sapiens
tgtgtggttctccttgcatcaggaggaagctacatacctacattt

SEQ ID NO: 916 - DNA, 45 bp, Homo sapiens
tgtgtggtgcgaatggcatcaggaggaagctacatacctacattt

SEQ ID NO: 917 - DNA, 45 bp, Homo sapiens
tgtgtggtgagatatgcatcaggaggaagctacatacctacattt

SEQ ID NO: 918 - DNA, 45 bp, Homo sapiens
tgtgtggttatcccggcatcaggaggaagctacatacctacattt

SEQ ID NO: 919 - DNA, 45 bp, Homo sapiens
tgtgtggtgaggcgtgcggcaggaggaagctacatacctacattt

SEQ ID NO: 920 - DNA, 45 bp, Homo sapiens
tgtgtggtgcctgaagcatcaggaggaagctacatacctacattt

SEQ ID NO: 921 - DNA, 45 bp, Homo sapiens
tgtgtggtgggccgggcatcaggaggaagctacatacctacattt

SEQ ID NO: 922 - DNA, 45 bp, Homo sapiens
tgtgtggtgatgcgagcctcaggaggaagctacatacctacattt

SEQ ID NO: 923 - DNA, 45 bp, Homo sapiens
tgtgtggtgaacggggcctcaggaggaagctacatacctacattt

SEQ ID NO: 924 - DNA, 45 bp, Homo sapiens
tgtgtggtgaaggaggcatcaggaggaagctacatacctacattt

SEQ ID NO: 925 - DNA, 45 bp, Homo sapiens
tgtgtggtaccccatgcatcaggaggaagctacatacctacattt

SEQ ID NO: 926 - DNA, 45 bp, Homo sapiens
tgtgtggtgaacagcgcgggaggaggaagctacatacctacattt

SEQ ID NO: 927 - DNA, 45 bp, Homo sapiens
tgtgtggtgatccgagcatcaggaggaagctacatacctacattt

SEQ ID NO: 928 - DNA, 45 bp, Homo sapiens
tgtgtggtgaccgaggcgtcaggaggaagctacatacctacattt

SEQ ID NO: 929 - DNA, 45 bp, Homo sapiens
tgtgtggtgaaatctgcatcaggaggaagctacatacctacattt

SEQ ID NO: 930 - DNA, 45 bp, Homo sapiens
tgtgtggtgaacggggcggcaggaggaagctacatacctacattt

SEQ ID NO: 931 - DNA, 45 bp, Homo sapiens
tgtgtggtgagcagggcatcaggaggaagctacatacctacattt

SEQ ID NO: 932 - DNA, 45 bp, Homo sapiens
tgtgtggtgaaccccgcctcaggaggaagctacatacctacattt

SEQ ID NO: 933 - DNA, 45 bp, Homo sapiens
tgtgtggtgaacagtgcgtcaggaggaagctacatacctacattt

SEQ ID NO: 934 - DNA, 45 bp, Homo sapiens
tgtgtggtgaaggcggcatcaggaggaagctacatacctacattt

SEQ ID NO: 935 - DNA, 45 bp, Homo sapiens
tgtgtggtgcccaccgcatcaggaggaagctacatacctacattt

SEQ ID NO: 936 - DNA, 45 bp, Homo sapiens
tgtgtggtccgcgaggcttcaggaggaagctacatacctacattt

SEQ ID NO: 937 - DNA, 45 bp, Homo sapiens
tgtgtggtggcccatgcatcaggaggaagctacatacctacattt

SEQ ID NO: 938 - DNA, 45 bp, Homo sapiens
tgtgtggtgattggagcatcaggaggaagctacatacctacattt

SEQ ID NO: 939 - DNA, 45 bp, Homo sapiens
tgtgtggtgaccggggcggcaggaggaagctacatacctacattt

SEQ ID NO: 940 - DNA, 45 bp, Homo sapiens
tgtgtggtgagcgatgcatcaggaggaagctacatacctacattt

SEQ ID NO: 941 - DNA, 45 bp, Homo sapiens
tgtgtggtgacgttggcgggaggaggaagctacatacctacattt

SEQ ID NO: 942 - DNA, 45 bp, Homo sapiens
tgtgtggtgaacatggcggaaggaggaagctacatacctacattt

SEQ ID NO: 943 - DNA, 45 bp, Homo sapiens
tgtgtggtgagtttagcatcaggaggaagctacatacctacattt

SEQ ID NO: 944 - DNA, 45 bp, Homo sapiens
tgtgtggtgaggaccgccaggggaggaagctacatacctacattt

SEQ ID NO: 945 - DNA, 45 bp, Homo sapiens
tgtgtggtgtctaaagcatcaggaggaagctacatacctacattt

SEQ ID NO: 946 - DNA, 45 bp, Homo sapiens
tgtgtggtgagtgtcgcatcaggaggaagctacatacctacattt

SEQ ID NO: 947 - DNA, 45 bp, Homo sapiens
tgtgtggtcccctccgcatcaggaggaagctacatacctacattt

SEQ ID NO: 948 - DNA, 45 bp, Homo sapiens
tgtgtggtccagctcgcatcaggaggaagctacatacctacattt

SEQ ID NO: 949 - DNA, 45 bp, Homo sapiens
tgtgtggtgagtacggcatcaggaggaagctacatacctacattt

SEQ ID NO: 950 - DNA, 45 bp, Homo sapiens
tgtgtggtgaggatggcatcaggaggaagctacatacctacattt

SEQ ID NO: 951 - DNA, 45 bp, Homo sapiens
tgtgtggtgagaatggcatcaggaggaagctacatacctacattt

SEQ ID NO: 952 - DNA, 45 bp, Homo sapiens
tgtgtggtgaactcagccgcaggaggaagctacatacctacattt

SEQ ID NO: 953 - DNA, 45 bp, Homo sapiens
tgtgtggtgaacatcgcagcaggaggaagctacatacctacattt

SEQ ID NO: 954 - DNA, 45 bp, Homo sapiens
tgtgtggtgcggaccgcttcaggaggaagctacatacctacattt

SEQ ID NO: 955 - DNA, 45 bp, Homo sapiens
tgtgtggtgcgacgagcatcaggaggaagctacatacctacattt

SEQ ID NO: 956 - DNA, 45 bp, Homo sapiens
tgtgtggtgagcatcgcatcaggaggaagctacatacctacattt

SEQ ID NO: 957 - DNA, 45 bp, Homo sapiens
tgtgtggtgtcccaggcggcaggaggaagctacatacctacattt

SEQ ID NO: 958 - DNA, 45 bp, Homo sapiens
tgtgtggtgtccctagcatcaggaggaagctacatacctacattt

SEQ ID NO: 959 - DNA, 45 bp, Homo sapiens
tgtgtggtgcacgtcgcatcaggaggaagctacatacctacattt

SEQ ID NO: 960 - DNA, 45 bp, Homo sapiens
tgtgtggtgatcgtcgcatcaggaggaagctacatacctacattt

SEQ ID NO: 961 - DNA, 45 bp, Homo sapiens
tgtgtggtgaccctcgccgggggaggaagctacatacctacattt

SEQ ID NO: 962 - DNA, 45 bp, Homo sapiens
tgtgtggtgaggcttgccgggggaggaagctacatacctacattt

SEQ ID NO: 963 - DNA, 45 bp, Homo sapiens
tgtgtggtgagtactgcatcaggaggaagctacatacctacattt

SEQ ID NO: 964 - DNA, 45 bp, Homo sapiens
tgtgtggtgaggtcggcctcaggaggaagctacatacctacattt

SEQ ID NO: 965 - DNA, 45 bp, Homo sapiens
tgtgtggtgaacgtcgcaacaggaggaagctacatacctacattt

SEQ ID NO: 966 - DNA, 45 bp, Homo sapiens
tgtgtggtgaacatggccgcaggaggaagctacatacctacattt

SEQ ID NO: 967 - DNA, 45 bp, Homo sapiens
tgtgtggtgaactcagcggcgggaggaagctacatacctacattt

SEQ ID NO: 968 - DNA, 45 bp, Homo sapiens
tgtgtggtgtttaccgcatcaggaggaagctacatacctacattt

SEQ ID NO: 969 - DNA, 45 bp, Homo sapiens
tgtgtggtgagaagtgcatcaggaggaagctacatacctacattt

SEQ ID NO: 970 - DNA, 45 bp, Homo sapiens
tgtgtggtgtccggggcatcaggaggaagctacatacctacattt

SEQ ID NO: 971 - DNA, 45 bp, Homo sapiens
tgtgtggtgaacgtcgcgacaggaggaagctacatacctacattt

SEQ ID NO: 972 - DNA, 45 bp, Homo sapiens
tgtgtggtttccctcgcatcaggaggaagctacatacctacattt

SEQ ID NO: 973 - DNA, 45 bp, Homo sapiens
tgtgtggtgtttgtggcatcaggaggaagctacatacctacattt

SEQ ID NO: 974 - DNA, 45 bp, Homo sapiens
tgtgtggtgacctatgcatcaggaggaagctacatacctacattt

SEQ ID NO: 975 - DNA, 45 bp, Homo sapiens
tgtgtggtttaccttgcatcaggaggaagctacatacctacattt

SEQ ID NO: 976 - DNA, 45 bp, Homo sapiens
tgtgtggtgaatgtcgcagggggaggaagctacatacctacattt

SEQ ID NO: 977 - DNA, 45 bp, Homo sapiens
tgtgtggtgaacatagccggaggaggaagctacatacctacattt

SEQ ID NO: 978 - DNA, 45 bp, Homo sapiens
tgtgtggtgaatgaagcatcaggaggaagctacatacctacattt

SEQ ID NO: 979 - DNA, 45 bp, Homo sapiens
tgtgtggtgatcctagcatcaggaggaagctacatacctacattt

SEQ ID NO: 980 - DNA, 45 bp, Homo sapiens
tgtgtggttgtctttgcatcaggaggaagctacatacctacattt

SEQ ID NO: 981 - DNA, 45 bp, Homo sapiens
tgtgtggtgaataaagcatcaggaggaagctacatacctacattt

SEQ ID NO: 982 - DNA, 45 bp, Homo sapiens
tgtgtggtgagacttgcatcaggaggaagctacatacctacattt

SEQ ID NO: 983 - DNA, 45 bp, Homo sapiens
tgtgtggtcgcccatgcatcaggaggaagctacatacctacattt

SEQ ID NO: 984 - DNA, 45 bp, Homo sapiens
tgtgtggtcaggtctgcatcaggaggaagctacatacctacattt

SEQ ID NO: 985 - DNA, 45 bp, Homo sapiens
tgtgtggtgccgaccgcatcaggaggaagctacatacctacattt

SEQ ID NO: 986 - DNA, 45 bp, Homo sapiens
tgtgtggtgcgtagtgcatcaggaggaagctacatacctacattt

SEQ ID NO: 987 - DNA, 45 bp, Homo sapiens
tgtgtggtgatcctagcttcaggaggaagctacatacctacattt

SEQ ID NO: 988 - DNA, 45 bp, Homo sapiens
tgtgtggtgcgacatgcatcaggaggaagctacatacctacattt

SEQ ID NO: 989 - DNA, 45 bp, Homo sapiens
tgtgtggttgcccatgcatcaggaggaagctacatacctacattt

SEQ ID NO: 990 - DNA, 45 bp, Homo sapiens
tgtgtggtgattcccgcctcaggaggaagctacatacctacattt

SEQ ID NO: 991 - DNA, 45 bp, Homo sapiens
tgtgtggtgacctccgcccgaggaggaagctacatacctacattt

SEQ ID NO: 992 - DNA, 45 bp, Homo sapiens
tgtgtggtgaacatcgcttcaggaggaagctacatacctacattt

SEQ ID NO: 993 - DNA, 45 bp, Homo sapiens
tgtgtggtgaacatcgccccaggaggaagctacatacctacattt

SEQ ID NO: 994 - DNA, 45 bp, Homo sapiens
tgtgtggtgaacagggccggaggaggaagctacatacctacattt

SEQ ID NO: 995 - DNA, 45 bp, Homo sapiens
tgtgtggtgaacaaggcctcaggaggaagctacatacctacattt

SEQ ID NO: 996 - DNA, 45 bp, Homo sapiens
tgtgtggtttttcatgcatcaggaggaagctacatacctacattt

SEQ ID NO: 997 - DNA, 45 bp, Homo sapiens
tgtgtggtgataagggcatcaggaggaagctacatacctacattt

SEQ ID NO: 998 - DNA, 45 bp, Homo sapiens
tgtgtggtgacccgtgcatcaggaggaagctacatacctacattt

SEQ ID NO: 999 - DNA, 45 bp, Homo sapiens
tgtgtggtgaacaacgcaagaggaggaagctacatacctacattt

SEQ ID NO: 1000 - DNA, 45 bp, Homo sapiens
tgtgtggtttcccgagcatcaggaggaagctacatacctacattt

SEQ ID NO: 1001 - DNA, 45 bp, Homo sapiens
tgtgtggtgaccgcggcatcaggaggaagctacatacctacattt

SEQ ID NO: 1002 - DNA, 45 bp, Homo sapiens
tgtgtggtgaacattgcggcaggaggaagctacatacctacattt

SEQ ID NO: 1003 - DNA, 45 bp, Homo sapiens
tgtgtggtcccccatgcatcaggaggaagctacatacctacattt

SEQ ID NO: 1004 - DNA, 45 bp, Homo sapiens
tgtgtggtgaacctcgcctcaggaggaagctacatacctacattt

SEQ ID NO: 1005 - DNA, 45 bp, Homo sapiens
tgtgtggtgcggggagcatcaggaggaagctacatacctacattt

SEQ ID NO: 1006 - DNA, 45 bp, Homo sapiens
tgtgtggtgccacatgcatcaggaggaagctacatacctacattt

SEQ ID NO: 1007 - DNA, 45 bp, Homo sapiens
tgtgtggtgccctctgcatcaggaggaagctacatacctacattt

SEQ ID NO: 1008 - DNA, 45 bp, Homo sapiens
tgtgtggtctccgttgcatcaggaggaagctacatacctacattt

SEQ ID NO: 1009 - DNA, 45 bp, Homo sapiens
tgtgtggtgagtggggcgcagggaggaagctacatacctacattt

SEQ ID NO: 1010 - DNA, 45 bp, Homo sapiens
tgtgtggttcgatccgcatcaggaggaagctacatacctacattt

SEQ ID NO: 1011 - DNA, 45 bp, Homo sapiens
tgtgtggtgagaaaagcatcaggaggaagctacatacctacattt

SEQ ID NO: 1012 - DNA, 45 bp, Homo sapiens
tgtgtggtgaacatcgcagaaggaggaagctacatacctacattt

SEQ ID NO: 1013 - DNA, 45 bp, Homo sapiens
tgtgtggtgagggctgcatcaggaggaagctacatacctacattt

SEQ ID NO: 1014 - DNA, 45 bp, Homo sapiens
tgtgtggtgaatatcgcatcaggaggaagctacatacctacattt

SEQ ID NO: 1015 - DNA, 45 bp, Homo sapiens
tgtgtggtgaagaccgcatcaggaggaagctacatacctacattt

SEQ ID NO: 1016 - DNA, 45 bp, Homo sapiens
tgtgtggtgaatagtgccgtaggaggaagctacatacctacattt

SEQ ID NO: 1017 - DNA, 45 bp, Homo sapiens
tgtgtggtgaggagggcatcaggaggaagctacatacctacattt

SEQ ID NO: 1018 - DNA, 45 bp, Homo sapiens
tgtgtggtgaacatggccggtggaggaagctacatacctacattt

SEQ ID NO: 1019 - DNA, 45 bp, Homo sapiens
tgtgtggtgggcacggcatcaggaggaagctacatacctacattt

SEQ ID NO: 1020 - DNA, 45 bp, Homo sapiens
tgtgtggtgagcagtgcatcaggaggaagctacatacctacattt

SEQ ID NO: 1021 - DNA, 45 bp, Homo sapiens
tgtgtggtgaacatggcgaggggaggaagctacatacctacattt

SEQ ID NO: 1022 - DNA, 45 bp, Homo sapiens
tgtgtggtgaaggttgcatcaggaggaagctacatacctacattt

SEQ ID NO: 1023 - DNA, 45 bp, Homo sapiens
tgtgtggtaaaacatgcatcaggaggaagctacatacctacattt

SEQ ID NO: 1024 - DNA, 45 bp, Homo sapiens
tgtgtggtcagagcggcatcaggaggaagctacatacctacattt

SEQ ID NO: 1025 - DNA, 45 bp, Homo sapiens
tgtgtggtgaacatggcagccggaggaagctacatacctacattt

SEQ ID NO: 1026 - DNA, 45 bp, Homo sapiens
tgtgtggtgagatccgcatcaggaggaagctacatacctacattt

SEQ ID NO: 1027 - DNA, 45 bp, Homo sapiens
tgtgtggtgaacatagcactcggaggaagctacatacctacattt

SEQ ID NO: 1028 - DNA, 45 bp, Homo sapiens
tgtgtggtgtcccaggcggggggaggaagctacatacctacattt

SEQ ID NO: 1029 - DNA, 45 bp, Homo sapiens
tgtgtggtgaccttggcggggggaggaagctacatacctacattt

SEQ ID NO: 1030 - DNA, 45 bp, Homo sapiens
tgtgtggtgagagtcgcatcaggaggaagctacatacctacattt

SEQ ID NO: 1031 - DNA, 45 bp, Homo sapiens
tgtgtggtgtctactgcatcaggaggaagctacatacctacattt

SEQ ID NO: 1032 - DNA, 45 bp, Homo sapiens
tgtgtggtgcgtttggccggggggggaagctacatacctacattt

SEQ ID NO: 1033 - DNA, 45 bp, Homo sapiens
tgtgtggtgcggactgcatcaggaggaagctacatacctacattt

SEQ ID NO: 1034 - DNA, 45 bp, Homo sapiens
tgtgtggtgaacgtcgcggccggaggaagctacatacctacattt

SEQ ID NO: 1035 - DNA, 45 bp, Homo sapiens
tgtgtggtggccgacgcatcaggaggaagctacatacctacattt

SEQ ID NO: 1036 - DNA, 45 bp, Homo sapiens
tgtgtggtgaacagggcgccaggaggaagctacatacctacattt

SEQ ID NO: 1037 - DNA, 45 bp, Homo sapiens
tgtgtggtgactctggcatcaggaggaagctacatacctacattt

SEQ ID NO: 1038 - DNA, 45 bp, Homo sapiens
tgtgtggtggttctcgcatcaggaggaagctacatacctacattt

SEQ ID NO: 1039 - DNA, 45 bp, Homo sapiens
tgtgtggtgaggggggcggagggaggaagctacatacctacattt

SEQ ID NO: 1040 - DNA, 45 bp, Homo sapiens
tgtgtggtgaacggggctacaggaggaagctacatacctacattt

SEQ ID NO: 1041 - DNA, 45 bp, Homo sapiens
tgtgtggtgtctgtagcatcaggaggaagctacatacctacattt

SEQ ID NO: 1042 - DNA, 45 bp, Homo sapiens
tgtgtggtgactccagcatcaggaggaagctacatacctacattt

SEQ ID NO: 1043 - DNA, 45 bp, Homo sapiens
tgtgtggtgatgggcgcatcaggaggaagctacatacctacattt

SEQ ID NO: 1044 - DNA, 45 bp, Homo sapiens
tgtgtggtgatccgcgcatcaggaggaagctacatacctacattt

SEQ ID NO: 1045 - DNA, 45 bp, Homo sapiens
tgtgtggtgagtgatgcatcaggaggaagctacatacctacattt

SEQ ID NO: 1046 - DNA, 45 bp, Homo sapiens
tgtgtggtccagcatgcatcaggaggaagctacatacctacattt

SEQ ID NO: 1047 - DNA, 45 bp, Homo sapiens
tgtgtggtgaagagggcctcaggaggaagctacatacctacattt

SEQ ID NO: 1048 - DNA, 45 bp, Homo sapiens
tgtgtggtcctcctcgcatcaggaggaagctacatacctacattt

SEQ ID NO: 1049 - DNA, 45 bp, Homo sapiens
tgtgtggtgatgggggcatcaggaggaagctacatacctacattt

SEQ ID NO: 1050 - DNA, 45 bp, Homo sapiens
tgtgtggtgaagagtgcatcaggaggaagctacatacctacattt

SEQ ID NO: 1051 - DNA, 45 bp, Homo sapiens
tgtgtggtggaccaagcatcaggaggaagctacatacctacattt

SEQ ID NO: 1052 - DNA, 45 bp, Homo sapiens
tgtgtggtgaactgggctgcaggaggaagctacatacctacattt

SEQ ID NO: 1053 - DNA, 45 bp, Homo sapiens
tgtgtggtgaaagatgcatcaggaggaagctacatacctacattt

SEQ ID NO: 1054 - DNA, 45 bp, Homo sapiens
tgtgtggtgtcccaagcatcaggaggaagctacatacctacattt

SEQ ID NO: 1055 - DNA, 45 bp, Homo sapiens
tgtgtggtgaacctcgcagcaggaggaagctacatacctacattt

SEQ ID NO: 1056 - DNA, 45 bp, Homo sapiens
tgtgtggtcacgggggcatcaggaggaagctacatacctacattt

SEQ ID NO: 1057 - DNA, 45 bp, Homo sapiens
tgtgtggtgaacgtcgcaccaggaggaagctacatacctacattt

SEQ ID NO: 1058 - DNA, 45 bp, Homo sapiens
tgtgtggtgattgcagcatcaggaggaagctacatacctacattt

SEQ ID NO: 1059 - DNA, 45 bp, Homo sapiens
tgtgtggtgatacatgcatcaggaggaagctacatacctacattt

SEQ ID NO: 1060 - DNA, 45 bp, Homo sapiens
tgtgtggtgaatccagcatcaggaggaagctacatacctacattt

SEQ ID NO: 1061 - DNA, 45 bp, Homo sapiens
tgtgtggtgaagcccgcatcaggaggaagctacatacctacattt

SEQ ID NO: 1062 - DNA, 45 bp, Homo sapiens
tgtgtggtgaagggggcaggaggaggaagctacatacctacattt

SEQ ID NO: 1063 - DNA, 45 bp, Homo sapiens
tgtgtggtgccgggggcatcaggaggaagctacatacctacattt

SEQ ID NO: 1064 - DNA, 45 bp, Homo sapiens
tgtgtggttttcggggcatcaggaggaagctacatacctacattt

SEQ ID NO: 1065 - DNA, 45 bp, Homo sapiens
tgtgtggtgtcccatgcctcaggaggaagctacatacctacattt

SEQ ID NO: 1066 - DNA, 45 bp, Homo sapiens
tgtgtggtggccgtagcatcaggaggaagctacatacctacattt

SEQ ID NO: 1067 - DNA, 45 bp, Homo sapiens
tgtgtggtgacccttgcagggggaggaagctacatacctacattt

SEQ ID NO: 1068 - DNA, 45 bp, Homo sapiens
tgtgtggtgacaaacgcaccaggaggaagctacatacctacattt

SEQ ID NO: 1069 - DNA, 45 bp, Homo sapiens
tgtgtggtgaacttggccgtgggaggaagctacatacctacattt

SEQ ID NO: 1070 - DNA, 45 bp, Homo sapiens
tgtgtggtgaacgctgcagcaggaggaagctacatacctacattt

SEQ ID NO: 1071 - DNA, 45 bp, Homo sapiens
tgtgtggtgaacacagcatcaggaggaagctacatacctacattt

SEQ ID NO: 1072 - DNA, 45 bp, Homo sapiens
tgtgtggtgaatcccgcatcaggaggaagctacatacctacattt

SEQ ID NO: 1073 - DNA, 45 bp, Homo sapiens
tgtgtggtcctccctgcatcaggaggaagctacatacctacattt

SEQ ID NO: 1074 - DNA, 45 bp, Homo sapiens
tgtgtggtgagggacgcatcaggaggaagctacatacctacattt

SEQ ID NO: 1075 - DNA, 45 bp, Homo sapiens
tgtgtggtgacggctgcatcaggaggaagctacatacctacattt

SEQ ID NO: 1076 - DNA, 45 bp, Homo sapiens
tgtgtggtccacgatgcatcaggaggaagctacatacctacattt

SEQ ID NO: 1077 - DNA, 45 bp, Homo sapiens
tgtgtggtgatcgttgcatcaggaggaagctacatacctacattt

SEQ ID NO: 1078 - DNA, 45 bp, Homo sapiens
tgtgtggtgaaccttgccgcaggaggaagctacatacctacattt

SEQ ID NO: 1079 - DNA, 45 bp, Homo sapiens
tgtgtggtgaacgaagcttcaggaggaagctacatacctacattt

SEQ ID NO: 1080 - DNA, 45 bp, Homo sapiens
tgtgtggtgattttagcatcaggaggaagctacatacctacattt

SEQ ID NO: 1081 - DNA, 45 bp, Homo sapiens
tgtgtggtgactgtcgcatcaggaggaagctacatacctacattt

SEQ ID NO: 1082 - DNA, 45 bp, Homo sapiens
tgtgtggtgaacatcgcccgcggaggaagctacatacctacattt

SEQ ID NO: 1083 - DNA, 45 bp, Homo sapiens
tgtgtggtgaacatagccccaggaggaagctacatacctacattt

SEQ ID NO: 1084 - DNA, 45 bp, Homo sapiens
tgtgtggtgaacattgcagcaggaggaagctacatacctacattt

SEQ ID NO: 1085 - DNA, 45 bp, Homo sapiens
tgtgtggtgaacccggcaacaggaggaagctacatacctacattt

SEQ ID NO: 1086 - DNA, 45 bp, Homo sapiens
tgtgtggtgaacaaggcagcaggaggaagctacatacctacattt

SEQ ID NO: 1087 - DNA, 45 bp, Homo sapiens
tgtgtggtgaaacctgcatcaggaggaagctacatacctacattt

SEQ ID NO: 1088 - DNA, 45 bp, Homo sapiens
tgtgtggttggggtggcggcaggaggaagctacatacctacattt

SEQ ID NO: 1089 - DNA, 45 bp, Homo sapiens
tgtgtggtctatctagcatcaggaggaagctacatacctacattt

SEQ ID NO: 1090 - DNA, 45 bp, Homo sapiens
tgtgtggtgtctcatgcatcaggaggaagctacatacctacattt

SEQ ID NO: 1091 - DNA, 45 bp, Homo sapiens
tgtgtggtggcacatgcatcaggaggaagctacatacctacattt

SEQ ID NO: 1092 - DNA, 45 bp, Homo sapiens
tgtgtggttcttcatgcatcaggaggaagctacatacctacattt

SEQ ID NO: 1093 - DNA, 45 bp, Homo sapiens
tgtgtggtgaccggagcatcaggaggaagctacatacctacattt

SEQ ID NO: 1094 - DNA, 45 bp, Homo sapiens
tgtgtggtgaatgatgcatcaggaggaagctacatacctacattt

SEQ ID NO: 1095 - DNA, 45 bp, Homo sapiens
tgtgtggtgaactccgccacaggaggaagctacatacctacattt

SEQ ID NO: 1096 - DNA, 45 bp, Homo sapiens
tgtgtggtgaagcttgcatcaggaggaagctacatacctacattt

SEQ ID NO: 1097 - DNA, 45 bp, Homo sapiens
tgtgtggtgatcatagcctcaggaggaagctacatacctacattt

SEQ ID NO: 1098 - DNA, 45 bp, Homo sapiens
tgtgtggtgtcctccgcatcaggaggaagctacatacctacattt

SEQ ID NO: 1099 - DNA, 45 bp, Homo sapiens
tgtgtggtgatttcagcatcaggaggaagctacatacctacattt

SEQ ID NO: 1100 - DNA, 45 bp, Homo sapiens
tgtgtggtgagcgctgcatcaggaggaagctacatacctacattt

SEQ ID NO: 1101 - DNA, 45 bp, Homo sapiens
tgtgtggtgaagggggcatcaggaggaagctacatacctacattt

SEQ ID NO: 1102 - DNA, 45 bp, Homo sapiens
tgtgtggtgaaccgtgccccaggaggaagctacatacctacattt

SEQ ID NO: 1103 - DNA, 45 bp, Homo sapiens
tgtgtggtgaagtacgcatcaggaggaagctacatacctacattt

SEQ ID NO: 1104 - DNA, 45 bp, Homo sapiens
tgtgtggtggtacatgcatcaggaggaagctacatacctacattt

SEQ ID NO: 1105 - DNA, 45 bp, Homo sapiens
tgtgtggtcaacggggcatcaggaggaagctacatacctacattt

SEQ ID NO: 1106 - DNA, 45 bp, Homo sapiens
tgtgtggtgacacaggcatcaggaggaagctacatacctacattt

SEQ ID NO: 1107 - DNA, 45 bp, Homo sapiens
tgtgtggtgcccctggcgacaggaggaagctacatacctacattt

SEQ ID NO: 1108 - DNA, 45 bp, Homo sapiens
tgtgtggtgattcttgcatcaggaggaagctacatacctacattt

SEQ ID NO: 1109 - DNA, 45 bp, Homo sapiens
tgtgtggtgaacgaggcgggaggaggaagctacatacctacattt

SEQ ID NO: 1110 - DNA, 45 bp, Homo sapiens
tgtgtggtgattcccgcatcaggaggaagctacatacctacattt

SEQ ID NO: 1111 - DNA, 45 bp, Homo sapiens
tgtgtggtgattgcggcatcaggaggaagctacatacctacattt

SEQ ID NO: 1112 - DNA, 45 bp, Homo sapiens
tgtgtggtgcgggttgcatcaggaggaagctacatacctacattt

SEQ ID NO: 1113 - DNA, 45 bp, Homo sapiens
tgtgtggtgaacagggccccaggaggaagctacatacctacattt

SEQ ID NO: 1114 - DNA, 45 bp, Homo sapiens
tgtgtggtggagcaagcatcaggaggaagctacatacctacattt

SEQ ID NO: 1115 - DNA, 45 bp, Homo sapiens
tgtgtggtccgggcggcatcaggaggaagctacatacctacattt

SEQ ID NO: 1116 - DNA, 45 bp, Homo sapiens
tgtgtggtctacatggccccgggaggaagctacatacctacattt

SEQ ID NO: 1117 - DNA, 45 bp, Homo sapiens
tgtgtggtccgcatagcatcaggaggaagctacatacctacattt

SEQ ID NO: 1118 - DNA, 45 bp, Homo sapiens
tgtgtggtgatcttcgcatcaggaggaagctacatacctacattt

SEQ ID NO: 1119 - DNA, 45 bp, Homo sapiens
tgtgtggtgtcccgtgcatcaggaggaagctacatacctacattt

SEQ ID NO: 1120 - DNA, 45 bp, Homo sapiens
tgtgtggtgcgtggggcatcaggaggaagctacatacctacattt

SEQ ID NO: 1121 - DNA, 45 bp, Homo sapiens
tgtgtggtgactgttgcatcaggaggaagctacatacctacattt

SEQ ID NO: 1122 - DNA, 45 bp, Homo sapiens
tgtgtggtgtccgttgcatcaggaggaagctacatacctacattt

SEQ ID NO: 1123 - DNA, 45 bp, Homo sapiens
tgtgtggtgaacatcgcaggaggaggaagctacatacctacattt

SEQ ID NO: 1124 - DNA, 45 bp, Homo sapiens
tgtgtggtccggggggcatcaggaggaagctacatacctacattt

SEQ ID NO: 1125 - DNA, 45 bp, Homo sapiens
tgtgtggtatttcatgcatcaggaggaagctacatacctacattt

SEQ ID NO: 1126 - DNA, 45 bp, Homo sapiens
tgtgtggtgagccctgcatcaggaggaagctacatacctacattt

SEQ ID NO: 1127 - DNA, 45 bp, Homo sapiens
tgtgtggtgtccaccgcatcaggaggaagctacatacctacattt

SEQ ID NO: 1128 - DNA, 45 bp, Homo sapiens
tgtgtggtgaacttggcgtcaggaggaagctacatacctacattt

SEQ ID NO: 1129 - DNA, 45 bp, Homo sapiens
tgtgtggtgaggagagcatcaggaggaagctacatacctacattt

SEQ ID NO: 1130 - DNA, 45 bp, Homo sapiens
tgtgtggtgagttcagcatcaggaggaagctacatacctacattt

SEQ ID NO: 1131 - DNA, 45 bp, Homo sapiens
tgtgtggttcgcctcgcatcaggaggaagctacatacctacattt

SEQ ID NO: 1132 - DNA, 45 bp, Homo sapiens
tgtgtggtgaacagggcggcaggaggaagctacatacctacattt

SEQ ID NO: 1133 - DNA, 45 bp, Homo sapiens
tgtgtggtgacgcctgcatcaggaggaagctacatacctacattt

SEQ ID NO: 1134 - DNA, 45 bp, Homo sapiens
tgtgtggtgaaccgggccacaggaggaagctacatacctacattt

SEQ ID NO: 1135 - DNA, 45 bp, Homo sapiens
tgtgtggtctccctagcgggaggaggaagctacatacctacattt

SEQ ID NO: 1136 - DNA, 45 bp, Homo sapiens
tgtgtggtgagccctgcttcaggaggaagctacatacctacattt

SEQ ID NO: 1137 - DNA, 45 bp, Homo sapiens
tgtgtggtgtctagtgcatcaggaggaagctacatacctacattt

SEQ ID NO: 1138 - DNA, 45 bp, Homo sapiens
tgtgtggtggcccttgcatcaggaggaagctacatacctacattt

SEQ ID NO: 1139 - DNA, 45 bp, Homo sapiens
tgtgtggtgatgcatgcatcaggaggaagctacatacctacattt

SEQ ID NO: 1140 - DNA, 45 bp, Homo sapiens
tgtgtggtgaaccaggcctcaggaggaagctacatacctacattt

SEQ ID NO: 1141 - DNA, 45 bp, Homo sapiens
tgtgtggttatgaaggcggaaggaggaagctacatacctacattt

SEQ ID NO: 1142 - DNA, 45 bp, Homo sapiens
tgtgtggtgaaccccgcttcaggaggaagctacatacctacattt

SEQ ID NO: 1143 - DNA, 45 bp, Homo sapiens
tgtgtggtgaacggagcagtaggaggaagctacatacctacattt

SEQ ID NO: 1144 - DNA, 45 bp, Homo sapiens
tgtgtggtccgttctgcatcaggaggaagctacatacctacattt

SEQ ID NO: 1145 - DNA, 45 bp, Homo sapiens
tgtgtggtgattaatgcatcaggaggaagctacatacctacattt

SEQ ID NO: 1146 - DNA, 45 bp, Homo sapiens
tgtgtggtgaccagtgcatcaggaggaagctacatacctacattt

SEQ ID NO: 1147 - DNA, 45 bp, Homo sapiens
tgtgtggtgagctcggcatcaggaggaagctacatacctacattt

SEQ ID NO: 1148 - DNA, 45 bp, Homo sapiens
tgtgtggttcccccggcatcaggaggaagctacatacctacattt

SEQ ID NO: 1149 - DNA, 45 bp, Homo sapiens
tgtgtggtccgtagggcatcaggaggaagctacatacctacattt

SEQ ID NO: 1150 - DNA, 45 bp, Homo sapiens
tgtgtggtgtcctcagcatcaggaggaagctacatacctacattt

SEQ ID NO: 1151 - DNA, 45 bp, Homo sapiens
tgtgtggtgagagtagcatcaggaggaagctacatacctacattt

SEQ ID NO: 1152 - DNA, 45 bp, Homo sapiens
tgtgtggtggcccaggcatcaggaggaagctacatacctacattt

SEQ ID NO: 1153 - DNA, 45 bp, Homo sapiens
tgtgtggtgtctctagcatcaggaggaagctacatacctacattt

SEQ ID NO: 1154 - DNA, 45 bp, Homo sapiens
tgtgtggtgaactctgcgacaggaggaagctacatacctacattt

SEQ ID NO: 1155 - DNA, 45 bp, Homo sapiens
tgtgtggtgagtgtggcatcaggaggaagctacatacctacattt

SEQ ID NO: 1156 - DNA, 45 bp, Homo sapiens
tgtgtggtgaacatcgccggaggaggaagctacatacctacattt

SEQ ID NO: 1157 - DNA, 45 bp, Homo sapiens
tgtgtggtgaacctcgcagggggaggaagctacatacctacattt

SEQ ID NO: 1158 - DNA, 45 bp, Homo sapiens
tgtgtggtgagcggggcatcaggaggaagctacatacctacattt

SEQ ID NO: 1159 - DNA, 45 bp, Homo sapiens
tgtgtggtgagaggggcatcaggaggaagctacatacctacattt

SEQ ID NO: 1160 - DNA, 45 bp, Homo sapiens
tgtgtggtgttccaggcctcaggaggaagctacatacctacattt

SEQ ID NO: 1161 - DNA, 45 bp, Homo sapiens
tgtgtggtgactgctgcatcaggaggaagctacatacctacattt

SEQ ID NO: 1162 - DNA, 45 bp, Homo sapiens
tgtgtggtgagagaagcctggggaggaagctacatacctacattt

SEQ ID NO: 1163 - DNA, 45 bp, Homo sapiens
tgtgtggtgaactccgcgggaggaggaagctacatacctacattt

SEQ ID NO: 1164 - DNA, 45 bp, Homo sapiens
tgtgtggtggtcctcgcatcaggaggaagctacatacctacattt

SEQ ID NO: 1165 - DNA, 45 bp, Homo sapiens
tgtgtggtgaatctggcatcaggaggaagctacatacctacattt

SEQ ID NO: 1166 - DNA, 45 bp, Homo sapiens
tgtgtggtgcgtttagcatcaggaggaagctacatacctacattt

SEQ ID NO: 1167 - DNA, 45 bp, Homo sapiens
tgtgtggtgaacgtcgcggcaggaggaagctacatacctacattt

SEQ ID NO: 1168 - DNA, 45 bp, Homo sapiens
tgtgtggtgaattcggcatcaggaggaagctacatacctacattt

SEQ ID NO: 1169 - DNA, 45 bp, Homo sapiens
tgtgtggtgaacgaagcctcaggaggaagctacatacctacattt

SEQ ID NO: 1170 - DNA, 45 bp, Homo sapiens
tgtgtggtgaggaaggcatcaggaggaagctacatacctacattt

SEQ ID NO: 1171 - DNA, 45 bp, Homo sapiens
tgtgtggtgaccccggcatcaggaggaagctacatacctacattt

SEQ ID NO: 1172 - DNA, 45 bp, Homo sapiens
tgtgtggtgaaagcggcagcaggaggaagctacatacctacattt

SEQ ID NO: 1173 - DNA, 45 bp, Homo sapiens
tgtgtggtgaacgatgcatcaggaggaagctacatacctacattt

SEQ ID NO: 1174 - DNA, 45 bp, Homo sapiens
tgtgtggtgaaccccgccctgggaggaagctacatacctacattt

SEQ ID NO: 1175 - DNA, 45 bp, Homo sapiens
tgtgtggtgaagctcgcatcaggaggaagctacatacctacattt

SEQ ID NO: 1176 - DNA, 45 bp, Homo sapiens
tgtgtggtgagacgggcatcaggaggaagctacatacctacattt

SEQ ID NO: 1177 - DNA, 45 bp, Homo sapiens
tgtgtggtgaacgaagcgtcaggaggaagctacatacctacattt

SEQ ID NO: 1178 - DNA, 45 bp, Homo sapiens
tgtgtggtggccggggcatcaggaggaagctacatacctacattt

SEQ ID NO: 1179 - DNA, 45 bp, Homo sapiens
tgtgtggtgagcggagcatcaggaggaagctacatacctacattt

SEQ ID NO: 1180 - DNA, 45 bp, Homo sapiens
tgtgtggtgaacgcggccccaggaggaagctacatacctacattt

SEQ ID NO: 1181 - DNA, 45 bp, Homo sapiens
tgtgtggtgcgggccgcatcaggaggaagctacatacctacattt

SEQ ID NO: 1182 - DNA, 45 bp, Homo sapiens
tgtgtggtgaacaccgcgtcaggaggaagctacatacctacattt

SEQ ID NO: 1183 - DNA, 45 bp, Homo sapiens
tgtgtggtgaggcgagcatcaggaggaagctacatacctacattt

SEQ ID NO: 1184 - DNA, 45 bp, Homo sapiens
tgtgtggtctccggggcatcaggaggaagctacatacctacattt

SEQ ID NO: 1185 - DNA, 45 bp, Homo sapiens
tgtgtggtgaagactgcatcaggaggaagctacatacctacattt

SEQ ID NO: 1186 - DNA, 45 bp, Homo sapiens
tgtgtggtgaccggggcatcaggaggaagctacatacctacattt

SEQ ID NO: 1187 - DNA, 45 bp, Homo sapiens
tgtgtggtgaacccggcgtcaggaggaagctacatacctacattt

SEQ ID NO: 1188 - DNA, 45 bp, Homo sapiens
tgtgtggtgaacaatgcaccaggaggaagctacatacctacattt

SEQ ID NO: 1189 - DNA, 45 bp, Homo sapiens
tgtgtggtgactcctgcatcaggaggaagctacatacctacattt

SEQ ID NO: 1190 - DNA, 45 bp, Homo sapiens
tgtgtggtgaatggggccgcaggaggaagctacatacctacattt

SEQ ID NO: 1191 - DNA, 45 bp, Homo sapiens
tgtgtggtgaatcaggcatcaggaggaagctacatacctacattt

SEQ ID NO: 1192 - DNA, 45 bp, Homo sapiens
tgtgtggtgagttttgcatcaggaggaagctacatacctacattt

SEQ ID NO: 1193 - DNA, 45 bp, Homo sapiens
tgtgtggtgaaccccgcgacaggaggaagctacatacctacattt

SEQ ID NO: 1194 - DNA, 45 bp, Homo sapiens
tgtgtggtccgcgaagcatcaggaggaagctacatacctacattt

SEQ ID NO: 1195 - DNA, 45 bp, Homo sapiens
tgtgtggtgatctttgcatcaggaggaagctacatacctacattt

SEQ ID NO: 1196 - DNA, 45 bp, Homo sapiens
tgtgtggtgacacacgcatcaggaggaagctacatacctacattt

SEQ ID NO: 1197 - DNA, 45 bp, Homo sapiens
tgtgtggtcactcatgcatcaggaggaagctacatacctacattt

SEQ ID NO: 1198 - DNA, 45 bp, Homo sapiens
tgtgtggtgaaggtagcatcaggaggaagctacatacctacattt

SEQ ID NO: 1199 - DNA, 45 bp, Homo sapiens
tgtgtggtgaacatcgcaacaggaggaagctacatacctacattt

SEQ ID NO: 1200 - DNA, 45 bp, Homo sapiens
tgtgtggtgttccaggcgaggggaggaagctacatacctacattt

SEQ ID NO: 1201 - DNA, 45 bp, Homo sapiens
tgtgtggtgaatggagcatcaggaggaagctacatacctacattt

SEQ ID NO: 1202 - DNA, 45 bp, Homo sapiens
tgtgtggtcccccttgcatcaggaggaagctacatacctacattt

SEQ ID NO: 1203 - DNA, 45 bp, Homo sapiens
tgtgtggtgagtatggcatcaggaggaagctacatacctacattt

SEQ ID NO: 1204 - DNA, 45 bp, Homo sapiens
tgtgtggtgaaaggtgcatcaggaggaagctacatacctacattt

SEQ ID NO: 1205 - DNA, 45 bp, Homo sapiens
tgtgtggtgatcagtgccccaggaggaagctacatacctacattt